European Patent Specification EP 4 071 159 B1, published December 13, 2023. Title: CRISSCROSS COOPERATIVE SELF-ASSEMBLY. Applicant: President and Fellows of Harvard College Dana-Farber Cancer Institute, Inc. Application Not Yet Assigned. The sequence listing filed with the application follows.

SEQUENCE LISTING (688 sequences)

SEQ ID NO: 1 - DNA, 42 bp, Artificial Sequence
  Synthetic Polynucleotide
atctgaactcgctacggcggggggagcccccgatttagagct

SEQ ID NO: 2 - DNA, 42 bp, Artificial Sequence
  Synthetic Polynucleotide
cattgctgataccgtttagctaacaaacatcaagaaaacaaa

SEQ ID NO: 3 - DNA, 42 bp, Artificial Sequence
  Synthetic Polynucleotide
gatacttgccctctctgtacataattaattttcccttagaat

SEQ ID NO: 4 - DNA, 42 bp, Artificial Sequence
  Synthetic Polynucleotide
gattgggcgttatcaatgttgttttgtcacaatcaatagaaa

SEQ ID NO: 5 - DNA, 42 bp, Artificial Sequence
  Synthetic Polynucleotide
tctaatgaagacaaatccccacgtcaccgacttgagccattt

SEQ ID NO: 6 - DNA, 42 bp, Artificial Sequence
  Synthetic Polynucleotide
aaacatcgggttgagtattatgtggcgagaaaggaagggaag

SEQ ID NO: 7 - DNA, 42 bp, Artificial Sequence
  Synthetic Polynucleotide
cgctggcattcgcatcaaaggcgaattattcatttcaattac

SEQ ID NO: 8 - DNA, 42 bp, Artificial Sequence
  Synthetic Polynucleotide
agtttataaatgagtatcaatttagattaagacgctgagaag

SEQ ID NO: 9 - DNA, 42 bp, Artificial Sequence
  Synthetic Polynucleotide
tatcgacatcattacgcatcgcaacatataaaagaaacgcaa

SEQ ID NO: 10 - DNA, 42 bp, Artificial Sequence
  Synthetic Polynucleotide
ccatgcagacatcacgaaggtcaccagtagcaccattaccat

SEQ ID NO: 11 - DNA, 42 bp, Artificial Sequence
  Synthetic Polynucleotide
aagataacgcttgtgaaaatgagggcgctggcaagtgtagcg

SEQ ID NO: 12 - DNA, 42 bp, Artificial Sequence
  Synthetic Polynucleotide
gctaacagtagggaaactgcggcctgattgctttgaatacca

SEQ ID NO: 13 - DNA, 42 bp, Artificial Sequence
  Synthetic Polynucleotide
atgggttcaggatgcaggtgaaatcataggtctgagagacta

SEQ ID NO: 14 - DNA, 42 bp, Artificial Sequence
  Synthetic Polynucleotide
ctcggatgggagtaagcgtatgcagtatgttagcaaacgtag

SEQ ID NO: 15 - DNA, 42 bp, Artificial Sequence
  Synthetic Polynucleotide
agagtttctgcggcagttaatcaatgaaaccatcgatagcag

SEQ ID NO: 16 - DNA, 42 bp, Artificial Sequence
  Synthetic Polynucleotide
gcaatacatcaaacgccgcgaacacccgccgcgcttaatgcg

SEQ ID NO: 17 - DNA, 42 bp, Artificial Sequence
  Synthetic Polynucleotide
tcaggcactgcgtgaagcggcagtaacagtaccttttacatc

SEQ ID NO: 18 - DNA, 42 bp, Artificial Sequence
  Synthetic Polynucleotide
atcaaaactcaacgagcagcggttgggttatataactatatg

SEQ ID NO: 19 - DNA, 42 bp, Artificial Sequence
  Synthetic Polynucleotide
agggttgtcggacttgtgcaaggaatacccaaaagaactggc

SEQ ID NO: 20 - DNA, 42 bp, Artificial Sequence
  Synthetic Polynucleotide
agtccgtgaagacggaaaccaaatcaagtttgcctttagcgt

SEQ ID NO: 21 - DNA, 42 bp, Artificial Sequence
  Synthetic Polynucleotide
ctggggatttgacgcagacctggttgctttgacgagcacgta

SEQ ID NO: 22 - DNA, 42 bp, Artificial Sequence
  Synthetic Polynucleotide
ttttcccagtcacgacgttgtgaaattgcgtagattttcagg

SEQ ID NO: 23 - DNA, 42 bp, Artificial Sequence
  Synthetic Polynucleotide
ttatcagtaaacagagaggtttcgcaagacaaagaacgcgag

SEQ ID NO: 24 - DNA, 42 bp, Artificial Sequence
  Synthetic Polynucleotide
tcagggattaatgaaagatggaacaaagttaccagaaggaaa

SEQ ID NO: 25 - DNA, 42 bp, Artificial Sequence
  Synthetic Polynucleotide
agtgtggcgatccgatagatgcggcattttcggtcatagccc

SEQ ID NO: 26 - DNA, 42 bp, Artificial Sequence
  Synthetic Polynucleotide
gggggatgtgctgcaaggcgaatcagagcgggagctaaacag

SEQ ID NO: 27 - DNA, 42 bp, Artificial Sequence
  Synthetic Polynucleotide
agccagctttccggcaccgctacctaccatatcaaaattatt

SEQ ID NO: 28 - DNA, 42 bp, Artificial Sequence
  Synthetic Polynucleotide
ctttattattcgcattcaccctagttaatttcatcttctgac

SEQ ID NO: 29 - DNA, 42 bp, Artificial Sequence
  Synthetic Polynucleotide
ttggtgtagatgggcgcatcgatcttaccgaagcccttttta

SEQ ID NO: 30 - DNA, 42 bp, Artificial Sequence
  Synthetic Polynucleotide
cagaaatagaagaattacagctttcataatcaaaatcaccgg

SEQ ID NO: 31 - DNA, 42 bp, Artificial Sequence
  Synthetic Polynucleotide
aagcgccattcgccattcaggagacaggaacggtacgccaga

SEQ ID NO: 32 - DNA, 42 bp, Artificial Sequence
  Synthetic Polynucleotide
tcagaaaagccccaaaaacagctgattgtttggattatactt

SEQ ID NO: 33 - DNA, 42 bp, Artificial Sequence
  Synthetic Polynucleotide
gaggggacgacgacagtatcgaccgaccgtgtgataaataag

SEQ ID NO: 34 - DNA, 42 bp, Artificial Sequence
  Synthetic Polynucleotide
tttttgttaaatcagctcattagcccaataataagagcaaga

SEQ ID NO: 35 - DNA, 42 bp, Artificial Sequence
  Synthetic Polynucleotide
gtgggaacaaacggcggattgcgcctccctcagagccgccac

SEQ ID NO: 36 - DNA, 42 bp, Artificial Sequence
  Synthetic Polynucleotide
tcgtaaaactagcatgtcaatatcagtgaggccaccgagtaa

SEQ ID NO: 37 - DNA, 42 bp, Artificial Sequence
  Synthetic Polynucleotide
atgatattcaaccgttctagcatattcctgattatcagatga

SEQ ID NO: 38 - DNA, 42 bp, Artificial Sequence
  Synthetic Polynucleotide
ttaaattgtaaacgttaatatcggaatcataattactagaaa

SEQ ID NO: 39 - DNA, 42 bp, Artificial Sequence
  Synthetic Polynucleotide
tattttaaatgcaatgcctgatgagcgctaatatcagagaga

SEQ ID NO: 40 - DNA, 42 bp, Artificial Sequence
  Synthetic Polynucleotide
tcaaaaataattcgcgtctggagccaccaccctcagagccgc

SEQ ID NO: 41 - DNA, 42 bp, Artificial Sequence
  Synthetic Polynucleotide
ggtagctatttttgagagatcattaaccgttgtagcaatact

SEQ ID NO: 42 - DNA, 42 bp, Artificial Sequence
  Synthetic Polynucleotide
atggtcaataacctgtttagcttgcggaacaaagaaaccacc

SEQ ID NO: 43 - DNA, 42 bp, Artificial Sequence
  Synthetic Polynucleotide
aaaagggtgagaaaggccggacgttatacaaattcttaccag

SEQ ID NO: 44 - DNA, 42 bp, Artificial Sequence
  Synthetic Polynucleotide
aacatccaataaatcatacaggggagaattaactgaacaccc

SEQ ID NO: 45 - DNA, 42 bp, Artificial Sequence
  Synthetic Polynucleotide
ctttatttcaacgcaaggatacgccgccagcattgacaggag

SEQ ID NO: 46 - DNA, 42 bp, Artificial Sequence
  Synthetic Polynucleotide
cgaacgagtagatttagtttgacttgcctgagtagaagaact

SEQ ID NO: 47 - DNA, 42 bp, Artificial Sequence
  Synthetic Polynucleotide
catttttgcggatggcttagaccgaacgttattaattttaaa

SEQ ID NO: 48 - DNA, 42 bp, Artificial Sequence
  Synthetic Polynucleotide
agctgaaaaggtggcatcaattagggcttaattgagaatcgc

SEQ ID NO: 49 - DNA, 42 bp, Artificial Sequence
  Synthetic Polynucleotide
agcttcaaagcgaaccagacctttacagagagaataacataa

SEQ ID NO: 50 - DNA, 42 bp, Artificial Sequence
  Synthetic Polynucleotide
attaagcaataaagcctcagaggccttgatattcacaaacaa

SEQ ID NO: 51 - DNA, 42 bp, Artificial Sequence
  Synthetic Polynucleotide
ctgtagctcaacatgttttaaaatatccagaacaatattacc

SEQ ID NO: 52 - DNA, 42 bp, Artificial Sequence
  Synthetic Polynucleotide
ggcttttgcaaaagaagttttagactttacaaacaattcgac

SEQ ID NO: 53 - DNA, 42 bp, Artificial Sequence
  Synthetic Polynucleotide
aggattagagagtacctttaagtaatttaggcagaggcattt

SEQ ID NO: 54 - DNA, 42 bp, Artificial Sequence
  Synthetic Polynucleotide
aatattcattgaatccccctcgaaacgattttttgtttaacg

SEQ ID NO: 55 - DNA, 42 bp, Artificial Sequence
  Synthetic Polynucleotide
aagaggaagcccgaaagacttaatggaaagcgcagtctctga

SEQ ID NO: 56 - DNA, 42 bp, Artificial Sequence
  Synthetic Polynucleotide
accctcgtttaccagacgacgaacgctcatggaaatacctac

SEQ ID NO: 57 - DNA, 42 bp, Artificial Sequence
  Synthetic Polynucleotide
taacggaacaacattattacaagagccgtcaatagataatac

SEQ ID NO: 58 - DNA, 42 bp, Artificial Sequence
  Synthetic Polynucleotide
atgtttagactggatagcgtcataaagtaccgacaaaaggta

SEQ ID NO: 59 - DNA, 42 bp, Artificial Sequence
  Synthetic Polynucleotide
tgaattaccttatgcgattttttacaaaataaacagccatat

SEQ ID NO: 60 - DNA, 42 bp, Artificial Sequence
  Synthetic Polynucleotide
aaacgagaatgaccataaatccatacatggcttttgatgata

SEQ ID NO: 61 - DNA, 42 bp, Artificial Sequence
  Synthetic Polynucleotide
agatttaggaataccacattcaaatggattatttacattggc

SEQ ID NO: 62 - DNA, 42 bp, Artificial Sequence
  Synthetic Polynucleotide
cgaggcgcagacggtcaatcagttatctaaaatatctttagg

SEQ ID NO: 63 - DNA, 42 bp, Artificial Sequence
  Synthetic Polynucleotide
gtcaggacgttgggaagaaaagacaataaacaacatgttcag

SEQ ID NO: 64 - DNA, 42 bp, Artificial Sequence
  Synthetic Polynucleotide
aggctggctgaccttcatcaataccaacgctaacgagcgtct

SEQ ID NO: 65 - DNA, 42 bp, Artificial Sequence
  Synthetic Polynucleotide
taaattgggcttgagatggttttttaacggggtcagtgcctt

SEQ ID NO: 66 - DNA, 42 bp, Artificial Sequence
  Synthetic Polynucleotide
tgtgtcgaaatccgcgacctgagtaataaaagggacattctg

SEQ ID NO: 67 - DNA, 42 bp, Artificial Sequence
  Synthetic Polynucleotide
tacgaaggcaccaacctaaaactggtcagttggcaaatcaac

SEQ ID NO: 68 - DNA, 42 bp, Artificial Sequence
  Synthetic Polynucleotide
ctttgaaagaggacagatgaatatcaacaatagataagtcct

SEQ ID NO: 69 - DNA, 42 bp, Artificial Sequence
  Synthetic Polynucleotide
gtagcaacggctacagaggcttagttgctattttgcacccag

SEQ ID NO: 70 - DNA, 42 bp, Artificial Sequence
  Synthetic Polynucleotide
gatattcattacccaaatcaacagttaatgccccctgcctat

SEQ ID NO: 71 - DNA, 42 bp, Artificial Sequence
  Synthetic Polynucleotide
ctaaaacactcatctttgaccctgacctgaaagcgtaagaat

SEQ ID NO: 72 - DNA, 42 bp, Artificial Sequence
  Synthetic Polynucleotide
cgaataataattttttcacgtatcaccttgctgaacctcaaa

SEQ ID NO: 73 - DNA, 42 bp, Artificial Sequence
  Synthetic Polynucleotide
atgaggaagtttccattaaacatcctaatttacgagcatgta

SEQ ID NO: 74 - DNA, 42 bp, Artificial Sequence
  Synthetic Polynucleotide
ttcgaggtgaatttcttaaacacctcccgacttgcgggaggt

SEQ ID NO: 75 - DNA, 42 bp, Artificial Sequence
  Synthetic Polynucleotide
ggatcgtcaccctcagcagcgacatgaaagtattaagaggct

SEQ ID NO: 76 - DNA, 42 bp, Artificial Sequence
  Synthetic Polynucleotide
tttcagcggagtgagaatagatgaatggctattagtctttaa

SEQ ID NO: 77 - DNA, 42 bp, Artificial Sequence
  Synthetic Polynucleotide
ctacaacgcctgtagcattccagtgccacgctgagagccagc

SEQ ID NO: 78 - DNA, 42 bp, Artificial Sequence
  Synthetic Polynucleotide
ctccaaaaggagcctttaattgtctttccttatcattccaag

SEQ ID NO: 79 - DNA, 42 bp, Artificial Sequence
  Synthetic Polynucleotide
cagagccaccaccctcattttaaggcttatccggtattctaa

SEQ ID NO: 80 - DNA, 42 bp, Artificial Sequence
  Synthetic Polynucleotide
ccgacaatgacaacaaccatctaggattagcggggttttgct

SEQ ID NO: 81 - DNA, 49 bp, Artificial Sequence
  Synthetic Polynucleotide
tcgtaaaactagcatgtcaatatcagtgaggccaccgagtaagaaaaac

SEQ ID NO: 82 - DNA, 49 bp, Artificial Sequence
  Synthetic Polynucleotide
atgatattcaaccgttctagcatattcctgattatcagatgaagagtcc

SEQ ID NO: 83 - DNA, 49 bp, Artificial Sequence
  Synthetic Polynucleotide
ttaaattgtaaacgttaatatcggaatcataattactagaaaaatagcc

SEQ ID NO: 84 - DNA, 49 bp, Artificial Sequence
  Synthetic Polynucleotide
tattttaaatgcaatgcctgatgagcgctaatatcagagagaatggtgg

SEQ ID NO: 85 - DNA, 49 bp, Artificial Sequence
  Synthetic Polynucleotide
tcaaaaataattcgcgtctggagccaccaccctcagagccgccggtcca

SEQ ID NO: 86 - DNA, 49 bp, Artificial Sequence
  Synthetic Polynucleotide
ggtagctatttttgagagatcattaaccgttgtagcaatactcggtcca

SEQ ID NO: 87 - DNA, 49 bp, Artificial Sequence
  Synthetic Polynucleotide
atggtcaataacctgtttagcttgcggaacaaagaaaccaccatggtgg

SEQ ID NO: 88 - DNA, 49 bp, Artificial Sequence
  Synthetic Polynucleotide
aaaagggtgagaaaggccggacgttatacaaattcttaccagaatagcc

SEQ ID NO: 89 - DNA, 49 bp, Artificial Sequence
  Synthetic Polynucleotide
aacatccaataaatcatacaggggagaattaactgaacacccagagtcc

SEQ ID NO: 90 - DNA, 49 bp, Artificial Sequence
  Synthetic Polynucleotide
ctttatttcaacgcaaggatacgccgccagcattgacaggaggaaaaac

SEQ ID NO: 91 - DNA, 52 bp, Artificial Sequence
  Synthetic Polynucleotide
tcgtaaaactagcatgtcaatatcagtgaggccaccgagtaagaaaaaccgt

SEQ ID NO: 92 - DNA, 52 bp, Artificial Sequence
  Synthetic Polynucleotide
atgatattcaaccgttctagcatattcctgattatcagatgaagagtccact

SEQ ID NO: 93 - DNA, 52 bp, Artificial Sequence
  Synthetic Polynucleotide
ttaaattgtaaacgttaatatcggaatcataattactagaaaaatagcccga

SEQ ID NO: 94 - DNA, 52 bp, Artificial Sequence
  Synthetic Polynucleotide
tattttaaatgcaatgcctgatgagcgctaatatcagagagaatggtggttc

SEQ ID NO: 95 - DNA, 52 bp, Artificial Sequence
  Synthetic Polynucleotide
tcaaaaataattcgcgtctggagccaccaccctcagagccgccggtccacgc

SEQ ID NO: 96 - DNA, 52 bp, Artificial Sequence
  Synthetic Polynucleotide
ggtagctatttttgagagatcattaaccgttgtagcaatactcggtccacgc

SEQ ID NO: 97 - DNA, 52 bp, Artificial Sequence
  Synthetic Polynucleotide
atggtcaataacctgtttagcttgcggaacaaagaaaccaccatggtggttc

SEQ ID NO: 98 - DNA, 52 bp, Artificial Sequence
  Synthetic Polynucleotide
aaaagggtgagaaaggccggacgttatacaaattcttaccagaatagcccga

SEQ ID NO: 99 - DNA, 52 bp, Artificial Sequence
  Synthetic Polynucleotide
aacatccaataaatcatacaggggagaattaactgaacacccagagtccact

SEQ ID NO: 100 - DNA, 52 bp, Artificial Sequence
  Synthetic Polynucleotide
ctttatttcaacgcaaggatacgccgccagcattgacaggaggaaaaaccgt

SEQ ID NO: 101 - DNA, 42 bp, Artificial Sequence
  Synthetic Polynucleotide
caatattacataacaatcctccatttgaattaccttttttaa

SEQ ID NO: 102 - DNA, 42 bp, Artificial Sequence
  Synthetic Polynucleotide
actgataccgtgcaaaattatcaaagacaaaagggcgacatt

SEQ ID NO: 103 - DNA, 42 bp, Artificial Sequence
  Synthetic Polynucleotide
cgtaacgatctaaagttttgtaacatcgccattaaaaatacc

SEQ ID NO: 104 - DNA, 42 bp, Artificial Sequence
  Synthetic Polynucleotide
gaacccatgtaccgtaacactcgcactcatcgagaacaagca

SEQ ID NO: 105 - DNA, 42 bp, Artificial Sequence
  Synthetic Polynucleotide
taccgccaccctcagaaccgccgtcgagagggttgatataag

SEQ ID NO: 106 - DNA, 42 bp, Artificial Sequence
  Synthetic Polynucleotide
tcattaaaggtgaattatcacttctgcaatgtgcgagaaatg

SEQ ID NO: 107 - DNA, 42 bp, Artificial Sequence
  Synthetic Polynucleotide
gggaattagagccagcaaaatgtttatgtagatgaaggtata

SEQ ID NO: 108 - DNA, 42 bp, Artificial Sequence
  Synthetic Polynucleotide
caccgtaatcagtagcgacaggtttcttgttgttcgccatcc

SEQ ID NO: 109 - DNA, 42 bp, Artificial Sequence
  Synthetic Polynucleotide
ccttattagcgtttgccatctgcaacacagcaataaaaatgc

SEQ ID NO: 110 - DNA, 42 bp, Artificial Sequence
  Synthetic Polynucleotide
cctcagaaccgccaccctcagccttcctgtagccagctttca

SEQ ID NO: 111 - DNA, 42 bp, Artificial Sequence
  Synthetic Polynucleotide
gttgaggcaggtcagacgattgcataaagctaaatcggttgt

SEQ ID NO: 112 - DNA, 42 bp, Artificial Sequence
  Synthetic Polynucleotide
atttaccgttccagtaagcgtaaaaatcaggtctttaccctg

SEQ ID NO: 113 - DNA, 42 bp, Artificial Sequence
  Synthetic Polynucleotide
gagtaacagtgcccgtataaacgtaacaaagctgctcattca

SEQ ID NO: 114 - DNA, 42 bp, Artificial Sequence
  Synthetic Polynucleotide
gagactcctcaagagaaggatgcccacgcataaccgatatat

SEQ ID NO: 115 - DNA, 42 bp, Artificial Sequence
  Synthetic Polynucleotide
tagcaagcaaatcagatatagcagggatagcaagcccaatag

SEQ ID NO: 116 - DNA, 42 bp, Artificial Sequence
  Synthetic Polynucleotide
gcttctgtaaatcgtcgctataaacatatagatgattaaacc

SEQ ID NO: 117 - DNA, 42 bp, Artificial Sequence
  Synthetic Polynucleotide
agtattaacaccgcctgcaacacagacagccctcatagttag

SEQ ID NO: 118 - DNA, 42 bp, Artificial Sequence
  Synthetic Polynucleotide
gcactaaatcggaaccctaaattttgttttatggagatgata

SEQ ID NO: 119 - DNA, 42 bp, Artificial Sequence
  Synthetic Polynucleotide
aaagcgaaaggagcgggcgctctgaatttcgcgtcgtcttca

SEQ ID NO: 120 - DNA, 42 bp, Artificial Sequence
  Synthetic Polynucleotide
ccgctacagggcgcgtactattttccatgaattggtaacacc

SEQ ID NO: 121 - DNA, 42 bp, Artificial Sequence
  Synthetic Polynucleotide
gaggccgattaaagggattttctgcgcaactgttgggaaggg

SEQ ID NO: 122 - DNA, 42 bp, Artificial Sequence
  Synthetic Polynucleotide
aagagtctgtccatcacgcaatacaaaggctatcaggtcatt

SEQ ID NO: 123 - DNA, 42 bp, Artificial Sequence
  Synthetic Polynucleotide
caaactatcggccttgctggtatatgcaactaaagtacggtg

SEQ ID NO: 124 - DNA, 42 bp, Artificial Sequence
  Synthetic Polynucleotide
attttgacgctcaatcgtctgaactaatgcagatacataacg

SEQ ID NO: 125 - DNA, 42 bp, Artificial Sequence
  Synthetic Polynucleotide
gccaacagagatagaacccttcccagcgattataccaagcgc

SEQ ID NO: 126 - DNA, 42 bp, Artificial Sequence
  Synthetic Polynucleotide
tgcgcgaactgatagccctaacgtctttccagacgttagtaa

SEQ ID NO: 127 - DNA, 40 bp, Artificial Sequence
  Synthetic Polynucleotide
caaagggcgaaaaaccaacagctgattgccctgcgccagg

SEQ ID NO: 128 - DNA, 40 bp, Artificial Sequence
  Synthetic Polynucleotide
agtccactattaaagaagagagttgcagcaagcaacgcgc

SEQ ID NO: 129 - DNA, 40 bp, Artificial Sequence
  Synthetic Polynucleotide
tagggttgagtgttgtgccccagcaggcgaaaacctgtcg

SEQ ID NO: 130 - DNA, 32 bp, Artificial Sequence
  Synthetic Polynucleotide
aatcccttataaatcagttccgaaatcggcaa

SEQ ID NO: 131 - DNA, 19 bp, Artificial Sequence
  Synthetic Polynucleotide
gtgagacgggcgtctatca

SEQ ID NO: 132 - DNA, 24 bp, Artificial Sequence
  Synthetic Polynucleotide
gtggtttttgtttcctgtgtgaaa

SEQ ID NO: 133 - DNA, 40 bp, Artificial Sequence
  Synthetic Polynucleotide
cgtattggtcaccgcctggccctgacgtggactccaacgt

SEQ ID NO: 134 - DNA, 24 bp, Artificial Sequence
  Synthetic Polynucleotide
ggggagagattccacacaacatac

SEQ ID NO: 135 - DNA, 40 bp, Artificial Sequence
  Synthetic Polynucleotide
gaatcggccggtccacgctggttttccagtttggaacaag

SEQ ID NO: 136 - DNA, 24 bp, Artificial Sequence
  Synthetic Polynucleotide
tgccagctgtgtaaagcctggggt

SEQ ID NO: 137 - DNA, 40 bp, Artificial Sequence
  Synthetic Polynucleotide
gtcgggaaatcctgtttgatggtgaaagaatagcccgaga

SEQ ID NO: 138 - DNA, 32 bp, Artificial Sequence
  Synthetic Polynucleotide
gttgcgctcactgcccaactcacattaattgc

SEQ ID NO: 139 - DNA, 19 bp, Artificial Sequence
  Synthetic Polynucleotide
gtcatagctcttttcacca

SEQ ID NO: 140 - DNA, 24 bp, Artificial Sequence
  Synthetic Polynucleotide
ttgttatccgctcacagcggtttg

SEQ ID NO: 141 - DNA, 24 bp, Artificial Sequence
  Synthetic Polynucleotide
gagccggaagcataaagcattaat

SEQ ID NO: 142 - DNA, 24 bp, Artificial Sequence
  Synthetic Polynucleotide
gcctaatgagtgagctgctttcca

SEQ ID NO: 143 - DNA, 42 bp, Artificial Sequence
  Synthetic Polynucleotide
aaaatacatacataaaggtggctattacggggttggaggtca

SEQ ID NO: 144 - DNA, 42 bp, Artificial Sequence
  Synthetic Polynucleotide
tagcaaggccggaaacgtcaccgaacaagacccgttagtaac

SEQ ID NO: 145 - DNA, 42 bp, Artificial Sequence
  Synthetic Polynucleotide
cagactgtagcgcgttttcataacgaagacgcctggtcgttc

SEQ ID NO: 146 - DNA, 42 bp, Artificial Sequence
  Synthetic Polynucleotide
aaccagagccaccaccggaacaccgtaatgggataggtcacg

SEQ ID NO: 147 - DNA, 42 bp, Artificial Sequence
  Synthetic Polynucleotide
caccagaaccaccaccagagcaaaatttttagaaccctcata

SEQ ID NO: 148 - DNA, 42 bp, Artificial Sequence
  Synthetic Polynucleotide
ataaatcctcattaaagccagcaaatatcgcgttttaattcg

SEQ ID NO: 149 - DNA, 42 bp, Artificial Sequence
  Synthetic Polynucleotide
caggagtgtactggtaataagtaatttcaactttaatcattg

SEQ ID NO: 150 - DNA, 42 bp, Artificial Sequence
  Synthetic Polynucleotide
ttcggaacctattattctgaaaaagacagcatcggaacgagg

SEQ ID NO: 151 - DNA, 42 bp, Artificial Sequence
  Synthetic Polynucleotide
cagtaccaggcggataagtgccaccctcagaaccgccaccct

SEQ ID NO: 152 - DNA, 42 bp, Artificial Sequence
  Synthetic Polynucleotide
attcatatggtttaccagcgctatcacgagtacggtggaaac

SEQ ID NO: 153 - DNA, 42 bp, Artificial Sequence
  Synthetic Polynucleotide
agacaccacggaataagtttatgcagatccggtgtcttgtct

SEQ ID NO: 154 - DNA, 42 bp, Artificial Sequence
  Synthetic Polynucleotide
atgattaagactccttattactgctaaactggaaagcaacga

SEQ ID NO: 155 - DNA, 42 bp, Artificial Sequence
  Synthetic Polynucleotide
ccgaggaaacgcaataataacgttgccaggaggatctggaac

SEQ ID NO: 156 - DNA, 42 bp, Artificial Sequence
  Synthetic Polynucleotide
agaaaagtaagcagatagccgcagacatcattgattcagcat

SEQ ID NO: 157 - DNA, 42 bp, Artificial Sequence
  Synthetic Polynucleotide
aacaatgaaatagcaatagcttaaccgtgcatctgccagttt

SEQ ID NO: 158 - DNA, 42 bp, Artificial Sequence
  Synthetic Polynucleotide
taacccacaagaattgagttattttaaccaataggaacgcca

SEQ ID NO: 159 - DNA, 42 bp, Artificial Sequence
  Synthetic Polynucleotide
tgaacaaagtcagagggtaatgtaatgtgtaggtaaagattc

SEQ ID NO: 160 - DNA, 42 bp, Artificial Sequence
  Synthetic Polynucleotide
aaacagggaagcgcattagacgcaaggcaaagaattagcaaa

SEQ ID NO: 161 - DNA, 42 bp, Artificial Sequence
  Synthetic Polynucleotide
tcaaaaatgaaaatagcagccggaagcaaactccaacaggtc

SEQ ID NO: 162 - DNA, 42 bp, Artificial Sequence
  Synthetic Polynucleotide
tatttatcccaatccaaataaaaatgctttaaacagttcaga

SEQ ID NO: 163 - DNA, 42 bp, Artificial Sequence
  Synthetic Polynucleotide
ttccagagcctaatttgccagaagaactggctcattatacca

SEQ ID NO: 164 - DNA, 42 bp, Artificial Sequence
  Synthetic Polynucleotide
ctacaattttatcctgaatctgagtaatcttgacaagaaccg

SEQ ID NO: 165 - DNA, 42 bp, Artificial Sequence
  Synthetic Polynucleotide
tttgaagccttaaatcaagatttgaggactaaagactttttc

SEQ ID NO: 166 - DNA, 42 bp, Artificial Sequence
  Synthetic Polynucleotide
gaacgcgaggcgttttagcgaagcttgataccgatagttgcg

SEQ ID NO: 167 - DNA, 42 bp, Artificial Sequence
  Synthetic Polynucleotide
ccttgaaaacatagcgatagcgagttagagtctgagcaaaaa

SEQ ID NO: 168 - DNA, 42 bp, Artificial Sequence
  Synthetic Polynucleotide
agtcaatagtgaatttatcaagtatctgcatatgatgtctga

SEQ ID NO: 169 - DNA, 42 bp, Artificial Sequence
  Synthetic Polynucleotide
cctttttaacctccggcttagtgagtattacgaaggtgttat

SEQ ID NO: 170 - DNA, 42 bp, Artificial Sequence
  Synthetic Polynucleotide
taaatgctgatgcaaatccaacgaagtgagcgaaattaactc

SEQ ID NO: 171 - DNA, 42 bp, Artificial Sequence
  Synthetic Polynucleotide
aaaactttttcaaatatattttcatgcgtattaaccaacagt

SEQ ID NO: 172 - DNA, 42 bp, Artificial Sequence
  Synthetic Polynucleotide
ctaaatttaatggtttgaaatgcctcaggaagatcgcactcc

SEQ ID NO: 173 - DNA, 42 bp, Artificial Sequence
  Synthetic Polynucleotide
gcgttaaataagaataaacactttgttaaaattcgcattaaa

SEQ ID NO: 174 - DNA, 42 bp, Artificial Sequence
  Synthetic Polynucleotide
aagcctgtttagtatcatatggacagtcaaatcaccatcaat

SEQ ID NO: 175 - DNA, 42 bp, Artificial Sequence
  Synthetic Polynucleotide
tataaagccaacgctcaacagtctactaatagtagtagcatt

SEQ ID NO: 176 - DNA, 42 bp, Artificial Sequence
  Synthetic Polynucleotide
catatttaacaacgccaacatttgctccttttgataagaggt

SEQ ID NO: 177 - DNA, 42 bp, Artificial Sequence
  Synthetic Polynucleotide
tcgagccagtaataagagaatcaatactgcggaatcgtcata

SEQ ID NO: 178 - DNA, 42 bp, Artificial Sequence
  Synthetic Polynucleotide
aagtaattctgtccagacgacatctacgttaataaaacgaac

SEQ ID NO: 179 - DNA, 42 bp, Artificial Sequence
  Synthetic Polynucleotide
ctaatgcagaacgcgcctgttcggtgtacagaccaggcgcat

SEQ ID NO: 180 - DNA, 42 bp, Artificial Sequence
  Synthetic Polynucleotide
gaacaagaaaaataatatcccgggtaaaatacgtaatgccac

SEQ ID NO: 181 - DNA, 42 bp, Artificial Sequence
  Synthetic Polynucleotide
gaaaccaatcaataatcggctgtatcggtttatcagcttgct

SEQ ID NO: 182 - DNA, 42 bp, Artificial Sequence
  Synthetic Polynucleotide
aacgggtattaaaccaagtacgagtttcgtcaccagtacaaa

SEQ ID NO: 183 - DNA, 42 bp, Artificial Sequence
  Synthetic Polynucleotide
attaattacatttaacaatttgcactcgcggggatttatttt

SEQ ID NO: 184 - DNA, 42 bp, Artificial Sequence
  Synthetic Polynucleotide
ctgagcaaaagaagatgatgagaaacgacatacattgcaagg

SEQ ID NO: 185 - DNA, 42 bp, Artificial Sequence
  Synthetic Polynucleotide
agttacaaaatcgcgcagaggagagtgagatcggttttgtaa

SEQ ID NO: 186 - DNA, 42 bp, Artificial Sequence
  Synthetic Polynucleotide
gggagaaacaataacggattctgttgagcttgaaacagcaaa

SEQ ID NO: 187 - DNA, 42 bp, Artificial Sequence
  Synthetic Polynucleotide
tttaacgtcagatgaatatacagagcaggcaatgcatgacga

SEQ ID NO: 188 - DNA, 42 bp, Artificial Sequence
  Synthetic Polynucleotide
tgcacgtaaaacagaaataaaaaaacgacggccagtgccaag

SEQ ID NO: 189 - DNA, 42 bp, Artificial Sequence
  Synthetic Polynucleotide
ctgaataatggaagggttagatctggtgccggaaaccaggca

SEQ ID NO: 190 - DNA, 42 bp, Artificial Sequence
  Synthetic Polynucleotide
tggcaattcatcaatataatcgaagattgtataagcaaatat

SEQ ID NO: 191 - DNA, 42 bp, Artificial Sequence
  Synthetic Polynucleotide
agaaggagcggaattatcatctgataaattaatgccggagag

SEQ ID NO: 192 - DNA, 42 bp, Artificial Sequence
  Synthetic Polynucleotide
agtttgagtaacattatcatttatattttcatttggggcgcg

SEQ ID NO: 193 - DNA, 42 bp, Artificial Sequence
  Synthetic Polynucleotide
aactcgtattaaatcctttgcgcttaattgctgaatataatg

SEQ ID NO: 194 - DNA, 42 bp, Artificial Sequence
  Synthetic Polynucleotide
atttgaggatttagaagtattgccagagggggtaatagtaaa

SEQ ID NO: 195 - DNA, 42 bp, Artificial Sequence
  Synthetic Polynucleotide
agcactaacaactaatagattggtagaaagattcatcagttg

SEQ ID NO: 196 - DNA, 42 bp, Artificial Sequence
  Synthetic Polynucleotide
agttgaaaggaattgaggaagtaagggaaccgaactgaccaa

SEQ ID NO: 197 - DNA, 42 bp, Artificial Sequence
  Synthetic Polynucleotide
tatcaaaccctcaatcaatatcgaaagaggcaaaagaataca

SEQ ID NO: 198 - DNA, 42 bp, Artificial Sequence
  Synthetic Polynucleotide
agcaaatgaaaaatctaaagctgaaaatctccaaaaaaaagg

SEQ ID NO: 199 - DNA, 42 bp, Artificial Sequence
  Synthetic Polynucleotide
tgacggggaaagccggcgaaccttactgtttctttacataaa

SEQ ID NO: 200 - DNA, 42 bp, Artificial Sequence
  Synthetic Polynucleotide
gtcacgctgcgcgtaaccaccccaggagaacgaggatattgc

SEQ ID NO: 201 - DNA, 42 bp, Artificial Sequence
  Synthetic Polynucleotide
taacgtgctttcctcgttagattaagttgggtaacgccaggg

SEQ ID NO: 202 - DNA, 42 bp, Artificial Sequence
  Synthetic Polynucleotide
atcctgagaagtgtttttatacatatgtaccccggttgataa

SEQ ID NO: 203 - DNA, 42 bp, Artificial Sequence
  Synthetic Polynucleotide
tctttgattagtaataacatcaccattagatacatttcgcaa

SEQ ID NO: 204 - DNA, 42 bp, Artificial Sequence
  Synthetic Polynucleotide
gccagccattgcaacaggaaaataaaaaccaaaatagcgaga

SEQ ID NO: 205 - DNA, 42 bp, Artificial Sequence
  Synthetic Polynucleotide
agattcaccagtcacacgaccctccatgttacttagccggaa

SEQ ID NO: 206 - DNA, 42 bp, Artificial Sequence
  Synthetic Polynucleotide
acgtggcacagacaatattttaaggaacaactaaaggaattg

SEQ ID NO: 207 - DNA, 49 bp, Artificial Sequence
  Synthetic Polynucleotide
atctgaactcgctacggcggggggagcccccgatttagagctcggtcca

SEQ ID NO: 208 - DNA, 49 bp, Artificial Sequence
  Synthetic Polynucleotide
cattgctgataccgtttagctaacaaacatcaagaaaacaaaatggtgg

SEQ ID NO: 209 - DNA, 49 bp, Artificial Sequence
  Synthetic Polynucleotide
gatacttgccctctctgtacataattaattttcccttagaataatagcc

SEQ ID NO: 210 - DNA, 49 bp, Artificial Sequence
  Synthetic Polynucleotide
gattgggcgttatcaatgttgttttgtcacaatcaatagaaaagagtcc

SEQ ID NO: 211 - DNA, 49 bp, Artificial Sequence
  Synthetic Polynucleotide
tctaatgaagacaaatccccacgtcaccgacttgagccatttgaaaaac

SEQ ID NO: 212 - DNA, 49 bp, Artificial Sequence
  Synthetic Polynucleotide
aaacatcgggttgagtattatgtggcgagaaaggaagggaaggaaaaac

SEQ ID NO: 213 - DNA, 49 bp, Artificial Sequence
  Synthetic Polynucleotide
cgctggcattcgcatcaaaggcgaattattcatttcaattacagagtcc

SEQ ID NO: 214 - DNA, 49 bp, Artificial Sequence
  Synthetic Polynucleotide
agtttataaatgagtatcaatttagattaagacgctgagaagaatagcc

SEQ ID NO: 215 - DNA, 49 bp, Artificial Sequence
  Synthetic Polynucleotide
tatcgacatcattacgcatcgcaacatataaaagaaacgcaaatggtgg

SEQ ID NO: 216 - DNA, 49 bp, Artificial Sequence
  Synthetic Polynucleotide
ccatgcagacatcacgaaggtcaccagtagcaccattaccatcggtcca

SEQ ID NO: 217 - DNA, 49 bp, Artificial Sequence
  Synthetic Polynucleotide
aagataacgcttgtgaaaatgagggcgctggcaagtgtagcgcggtcca

SEQ ID NO: 218 - DNA, 49 bp, Artificial Sequence
  Synthetic Polynucleotide
gctaacagtagggaaactgcggcctgattgctttgaataccaatggtgg

SEQ ID NO: 219 - DNA, 49 bp, Artificial Sequence
  Synthetic Polynucleotide
atgggttcaggatgcaggtgaaatcataggtctgagagactaaatagcc

SEQ ID NO: 220 - DNA, 49 bp, Artificial Sequence
  Synthetic Polynucleotide
ctcggatgggagtaagcgtatgcagtatgttagcaaacgtagagagtcc

SEQ ID NO: 221 - DNA, 49 bp, Artificial Sequence
  Synthetic Polynucleotide
agagtttctgcggcagttaatcaatgaaaccatcgatagcaggaaaaac

SEQ ID NO: 222 - DNA, 49 bp, Artificial Sequence
  Synthetic Polynucleotide
gcaatacatcaaacgccgcgaacacccgccgcgcttaatgcggaaaaac

SEQ ID NO: 223 - DNA, 49 bp, Artificial Sequence
  Synthetic Polynucleotide
tcaggcactgcgtgaagcggcagtaacagtaccttttacatcagagtcc

SEQ ID NO: 224 - DNA, 49 bp, Artificial Sequence
  Synthetic Polynucleotide
atcaaaactcaacgagcagcggttgggttatataactatatgaatagcc

SEQ ID NO: 225 - DNA, 49 bp, Artificial Sequence
  Synthetic Polynucleotide
agggttgtcggacttgtgcaaggaatacccaaaagaactggcatggtgg

SEQ ID NO: 226 - DNA, 49 bp, Artificial Sequence
  Synthetic Polynucleotide
agtccgtgaagacggaaaccaaatcaagtttgcctttagcgtcggtcca

SEQ ID NO: 227 - DNA, 49 bp, Artificial Sequence
  Synthetic Polynucleotide
ctggggatttgacgcagacctggttgctttgacgagcacgtacggtcca

SEQ ID NO: 228 - DNA, 49 bp, Artificial Sequence
  Synthetic Polynucleotide
ttttcccagtcacgacgttgtgaaattgcgtagattttcaggatggtgg

SEQ ID NO: 229 - DNA, 49 bp, Artificial Sequence
  Synthetic Polynucleotide
ttatcagtaaacagagaggtttcgcaagacaaagaacgcgagaatagcc

SEQ ID NO: 230 - DNA, 49 bp, Artificial Sequence
  Synthetic Polynucleotide
tcagggattaatgaaagatggaacaaagttaccagaaggaaaagagtcc

SEQ ID NO: 231 - DNA, 49 bp, Artificial Sequence
  Synthetic Polynucleotide
agtgtggcgatccgatagatgcggcattttcggtcatagcccgaaaaac

SEQ ID NO: 232 - DNA, 49 bp, Artificial Sequence
  Synthetic Polynucleotide
gggggatgtgctgcaaggcgaatcagagcgggagctaaacaggaaaaac

SEQ ID NO: 233 - DNA, 49 bp, Artificial Sequence
  Synthetic Polynucleotide
agccagctttccggcaccgctacctaccatatcaaaattattagagtcc

SEQ ID NO: 234 - DNA, 49 bp, Artificial Sequence
  Synthetic Polynucleotide
ctttattattcgcattcaccctagttaatttcatcttctgacaatagcc

SEQ ID NO: 235 - DNA, 49 bp, Artificial Sequence
  Synthetic Polynucleotide
ttggtgtagatgggcgcatcgatcttaccgaagccctttttaatggtgg

SEQ ID NO: 236 - DNA, 49 bp, Artificial Sequence
  Synthetic Polynucleotide
cagaaatagaagaattacagctttcataatcaaaatcaccggcggtcca

SEQ ID NO: 237 - DNA, 49 bp, Artificial Sequence
  Synthetic Polynucleotide
aagcgccattcgccattcaggagacaggaacggtacgccagacggtcca

SEQ ID NO: 238 - DNA, 49 bp, Artificial Sequence
  Synthetic Polynucleotide
tcagaaaagccccaaaaacagctgattgtttggattatacttatggtgg

SEQ ID NO: 239 - DNA, 49 bp, Artificial Sequence
  Synthetic Polynucleotide
gaggggacgacgacagtatcgaccgaccgtgtgataaataagaatagcc

SEQ ID NO: 240 - DNA, 49 bp, Artificial Sequence
  Synthetic Polynucleotide
tttttgttaaatcagctcattagcccaataataagagcaagaagagtcc

SEQ ID NO: 241 - DNA, 49 bp, Artificial Sequence
  Synthetic Polynucleotide
gtgggaacaaacggcggattgcgcctccctcagagccgccacgaaaaac

SEQ ID NO: 242 - DNA, 49 bp, Artificial Sequence
  Synthetic Polynucleotide
cgaacgagtagatttagtttgacttgcctgagtagaagaactgaaaaac

SEQ ID NO: 243 - DNA, 49 bp, Artificial Sequence
  Synthetic Polynucleotide
catttttgcggatggcttagaccgaacgttattaattttaaaagagtcc

SEQ ID NO: 244 - DNA, 49 bp, Artificial Sequence
  Synthetic Polynucleotide
agctgaaaaggtggcatcaattagggcttaattgagaatcgcaatagcc

SEQ ID NO: 245 - DNA, 49 bp, Artificial Sequence
  Synthetic Polynucleotide
agcttcaaagcgaaccagacctttacagagagaataacataaatggtgg

SEQ ID NO: 246 - DNA, 49 bp, Artificial Sequence
  Synthetic Polynucleotide
attaagcaataaagcctcagaggccttgatattcacaaacaacggtcca

SEQ ID NO: 247 - DNA, 49 bp, Artificial Sequence
  Synthetic Polynucleotide
ctgtagctcaacatgttttaaaatatccagaacaatattacccggtcca

SEQ ID NO: 248 - DNA, 49 bp, Artificial Sequence
  Synthetic Polynucleotide
ggcttttgcaaaagaagttttagactttacaaacaattcgacatggtgg

SEQ ID NO: 249 - DNA, 49 bp, Artificial Sequence
  Synthetic Polynucleotide
aggattagagagtacctttaagtaatttaggcagaggcatttaatagcc

SEQ ID NO: 250 - DNA, 49 bp, Artificial Sequence
  Synthetic Polynucleotide
aatattcattgaatccccctcgaaacgattttttgtttaacgagagtcc

SEQ ID NO: 251 - DNA, 49 bp, Artificial Sequence
  Synthetic Polynucleotide
aagaggaagcccgaaagacttaatggaaagcgcagtctctgagaaaaac

SEQ ID NO: 252 - DNA, 49 bp, Artificial Sequence
  Synthetic Polynucleotide
accctcgtttaccagacgacgaacgctcatggaaatacctacgaaaaac

SEQ ID NO: 253 - DNA, 49 bp, Artificial Sequence
  Synthetic Polynucleotide
taacggaacaacattattacaagagccgtcaatagataatacagagtcc

SEQ ID NO: 254 - DNA, 49 bp, Artificial Sequence
  Synthetic Polynucleotide
atgtttagactggatagcgtcataaagtaccgacaaaaggtaaatagcc

SEQ ID NO: 255 - DNA, 49 bp, Artificial Sequence
  Synthetic Polynucleotide
tgaattaccttatgcgattttttacaaaataaacagccatatatggtgg

SEQ ID NO: 256 - DNA, 49 bp, Artificial Sequence
  Synthetic Polynucleotide
aaacgagaatgaccataaatccatacatggcttttgatgatacggtcca

SEQ ID NO: 257 - DNA, 49 bp, Artificial Sequence
  Synthetic Polynucleotide
agatttaggaataccacattcaaatggattatttacattggccggtcca

SEQ ID NO: 258 - DNA, 49 bp, Artificial Sequence
  Synthetic Polynucleotide
cgaggcgcagacggtcaatcagttatctaaaatatctttaggatggtgg

SEQ ID NO: 259 - DNA, 49 bp, Artificial Sequence
  Synthetic Polynucleotide
gtcaggacgttgggaagaaaagacaataaacaacatgttcagaatagcc

SEQ ID NO: 260 - DNA, 49 bp, Artificial Sequence
  Synthetic Polynucleotide
aggctggctgaccttcatcaataccaacgctaacgagcgtctagagtcc

SEQ ID NO: 261 - DNA, 49 bp, Artificial Sequence
  Synthetic Polynucleotide
taaattgggcttgagatggttttttaacggggtcagtgccttgaaaaac

SEQ ID NO: 262 - DNA, 49 bp, Artificial Sequence
  Synthetic Polynucleotide
tgtgtcgaaatccgcgacctgagtaataaaagggacattctggaaaaac

SEQ ID NO: 263 - DNA, 49 bp, Artificial Sequence
  Synthetic Polynucleotide
tacgaaggcaccaacctaaaactggtcagttggcaaatcaacagagtcc

SEQ ID NO: 264 - DNA, 49 bp, Artificial Sequence
  Synthetic Polynucleotide
ctttgaaagaggacagatgaatatcaacaatagataagtcctaatagcc

SEQ ID NO: 265 - DNA, 49 bp, Artificial Sequence
  Synthetic Polynucleotide
gtagcaacggctacagaggcttagttgctattttgcacccagatggtgg

SEQ ID NO: 266 - DNA, 49 bp, Artificial Sequence
  Synthetic Polynucleotide
gatattcattacccaaatcaacagttaatgccccctgcctatcggtcca

SEQ ID NO: 267 - DNA, 49 bp, Artificial Sequence
  Synthetic Polynucleotide
ctaaaacactcatctttgaccctgacctgaaagcgtaagaatcggtcca

SEQ ID NO: 268 - DNA, 49 bp, Artificial Sequence
  Synthetic Polynucleotide
cgaataataattttttcacgtatcaccttgctgaacctcaaaatggtgg

SEQ ID NO: 269 - DNA, 49 bp, Artificial Sequence
  Synthetic Polynucleotide
atgaggaagtttccattaaacatcctaatttacgagcatgtaaatagcc

SEQ ID NO: 270 - DNA, 49 bp, Artificial Sequence
  Synthetic Polynucleotide
ttcgaggtgaatttcttaaacacctcccgacttgcgggaggtagagtcc

SEQ ID NO: 271 - DNA, 49 bp, Artificial Sequence
  Synthetic Polynucleotide
ggatcgtcaccctcagcagcgacatgaaagtattaagaggctgaaaaac

SEQ ID NO: 272 - DNA, 49 bp, Artificial Sequence
  Synthetic Polynucleotide
tttcagcggagtgagaatagatgaatggctattagtctttaagaaaaac

SEQ ID NO: 273 - DNA, 49 bp, Artificial Sequence
  Synthetic Polynucleotide
ctacaacgcctgtagcattccagtgccacgctgagagccagcagagtcc

SEQ ID NO: 274 - DNA, 49 bp, Artificial Sequence
  Synthetic Polynucleotide
ctccaaaaggagcctttaattgtctttccttatcattccaagaatagcc

SEQ ID NO: 275 - DNA, 49 bp, Artificial Sequence
  Synthetic Polynucleotide
cagagccaccaccctcattttaaggcttatccggtattctaaatggtgg

SEQ ID NO: 276 - DNA, 49 bp, Artificial Sequence
  Synthetic Polynucleotide
ccgacaatgacaacaaccatctaggattagcggggttttgctcggtcca

SEQ ID NO: 277 - DNA, 52 bp, Artificial Sequence
  Synthetic Polynucleotide
atctgaactcgctacggcggggggagcccccgatttagagctcggtccacgc

SEQ ID NO: 278 - DNA, 52 bp, Artificial Sequence
  Synthetic Polynucleotide
cattgctgataccgtttagctaacaaacatcaagaaaacaaaatggtggttc

SEQ ID NO: 279 - DNA, 52 bp, Artificial Sequence
  Synthetic Polynucleotide
gatacttgccctctctgtacataattaattttcccttagaataatagcccga

SEQ ID NO: 280 - DNA, 52 bp, Artificial Sequence
  Synthetic Polynucleotide
gattgggcgttatcaatgttgttttgtcacaatcaatagaaaagagtccact

SEQ ID NO: 281 - DNA, 52 bp, Artificial Sequence
  Synthetic Polynucleotide
tctaatgaagacaaatccccacgtcaccgacttgagccatttgaaaaaccgt

SEQ ID NO: 282 - DNA, 52 bp, Artificial Sequence
  Synthetic Polynucleotide
aaacatcgggttgagtattatgtggcgagaaaggaagggaaggaaaaaccgt

SEQ ID NO: 283 - DNA, 52 bp, Artificial Sequence
  Synthetic Polynucleotide
cgctggcattcgcatcaaaggcgaattattcatttcaattacagagtccact

SEQ ID NO: 284 - DNA, 52 bp, Artificial Sequence
  Synthetic Polynucleotide
agtttataaatgagtatcaatttagattaagacgctgagaagaatagcccga

SEQ ID NO: 285 - DNA, 52 bp, Artificial Sequence
  Synthetic Polynucleotide
tatcgacatcattacgcatcgcaacatataaaagaaacgcaaatggtggttc

SEQ ID NO: 286 - DNA, 52 bp, Artificial Sequence
  Synthetic Polynucleotide
ccatgcagacatcacgaaggtcaccagtagcaccattaccatcggtccacgc

SEQ ID NO: 287 - DNA, 52 bp, Artificial Sequence
  Synthetic Polynucleotide
aagataacgcttgtgaaaatgagggcgctggcaagtgtagcgcggtccacgc

SEQ ID NO: 288 - DNA, 52 bp, Artificial Sequence
  Synthetic Polynucleotide
gctaacagtagggaaactgcggcctgattgctttgaataccaatggtggttc

SEQ ID NO: 289 - DNA, 52 bp, Artificial Sequence
  Synthetic Polynucleotide
atgggttcaggatgcaggtgaaatcataggtctgagagactaaatagcccga

SEQ ID NO: 290 - DNA, 52 bp, Artificial Sequence
  Synthetic Polynucleotide
ctcggatgggagtaagcgtatgcagtatgttagcaaacgtagagagtccact

SEQ ID NO: 291 - DNA, 52 bp, Artificial Sequence
  Synthetic Polynucleotide
agagtttctgcggcagttaatcaatgaaaccatcgatagcaggaaaaaccgt

SEQ ID NO: 292 - DNA, 52 bp, Artificial Sequence
  Synthetic Polynucleotide
gcaatacatcaaacgccgcgaacacccgccgcgcttaatgcggaaaaaccgt

SEQ ID NO: 293 - DNA, 52 bp, Artificial Sequence
  Synthetic Polynucleotide
tcaggcactgcgtgaagcggcagtaacagtaccttttacatcagagtccact

SEQ ID NO: 294 - DNA, 52 bp, Artificial Sequence
  Synthetic Polynucleotide
atcaaaactcaacgagcagcggttgggttatataactatatgaatagcccga

SEQ ID NO: 295 - DNA, 52 bp, Artificial Sequence
  Synthetic Polynucleotide
agggttgtcggacttgtgcaaggaatacccaaaagaactggcatggtggttc

SEQ ID NO: 296 - DNA, 52 bp, Artificial Sequence
  Synthetic Polynucleotide
agtccgtgaagacggaaaccaaatcaagtttgcctttagcgtcggtccacgc

SEQ ID NO: 297 - DNA, 52 bp, Artificial Sequence
  Synthetic Polynucleotide
ctggggatttgacgcagacctggttgctttgacgagcacgtacggtccacgc

SEQ ID NO: 298 - DNA, 52 bp, Artificial Sequence
  Synthetic Polynucleotide
ttttcccagtcacgacgttgtgaaattgcgtagattttcaggatggtggttc

SEQ ID NO: 299 - DNA, 52 bp, Artificial Sequence
  Synthetic Polynucleotide
ttatcagtaaacagagaggtttcgcaagacaaagaacgcgagaatagcccga

SEQ ID NO: 300 - DNA, 52 bp, Artificial Sequence
  Synthetic Polynucleotide
tcagggattaatgaaagatggaacaaagttaccagaaggaaaagagtccact

SEQ ID NO: 301 - DNA, 52 bp, Artificial Sequence
  Synthetic Polynucleotide
agtgtggcgatccgatagatgcggcattttcggtcatagcccgaaaaaccgt

SEQ ID NO: 302 - DNA, 52 bp, Artificial Sequence
  Synthetic Polynucleotide
gggggatgtgctgcaaggcgaatcagagcgggagctaaacaggaaaaaccgt

SEQ ID NO: 303 - DNA, 52 bp, Artificial Sequence
  Synthetic Polynucleotide
agccagctttccggcaccgctacctaccatatcaaaattattagagtccact

SEQ ID NO: 304 - DNA, 52 bp, Artificial Sequence
  Synthetic Polynucleotide
ctttattattcgcattcaccctagttaatttcatcttctgacaatagcccga

SEQ ID NO: 305 - DNA, 52 bp, Artificial Sequence
  Synthetic Polynucleotide
ttggtgtagatgggcgcatcgatcttaccgaagccctttttaatggtggttc

SEQ ID NO: 306 - DNA, 52 bp, Artificial Sequence
  Synthetic Polynucleotide
cagaaatagaagaattacagctttcataatcaaaatcaccggcggtccacgc

SEQ ID NO: 307 - DNA, 52 bp, Artificial Sequence
  Synthetic Polynucleotide
aagcgccattcgccattcaggagacaggaacggtacgccagacggtccacgc

SEQ ID NO: 308 - DNA, 52 bp, Artificial Sequence
  Synthetic Polynucleotide
tcagaaaagccccaaaaacagctgattgtttggattatacttatggtggttc

SEQ ID NO: 309 - DNA, 52 bp, Artificial Sequence
  Synthetic Polynucleotide
gaggggacgacgacagtatcgaccgaccgtgtgataaataagaatagcccga

SEQ ID NO: 310 - DNA, 52 bp, Artificial Sequence
  Synthetic Polynucleotide
tttttgttaaatcagctcattagcccaataataagagcaagaagagtccact

SEQ ID NO: 311 - DNA, 52 bp, Artificial Sequence
  Synthetic Polynucleotide
gtgggaacaaacggcggattgcgcctccctcagagccgccacgaaaaaccgt

SEQ ID NO: 312 - DNA, 52 bp, Artificial Sequence
  Synthetic Polynucleotide
cgaacgagtagatttagtttgacttgcctgagtagaagaactgaaaaaccgt

SEQ ID NO: 313 - DNA, 52 bp, Artificial Sequence
  Synthetic Polynucleotide
catttttgcggatggcttagaccgaacgttattaattttaaaagagtccact

SEQ ID NO: 314 - DNA, 52 bp, Artificial Sequence
  Synthetic Polynucleotide
agctgaaaaggtggcatcaattagggcttaattgagaatcgcaatagcccga

SEQ ID NO: 315 - DNA, 52 bp, Artificial Sequence
  Synthetic Polynucleotide
agcttcaaagcgaaccagacctttacagagagaataacataaatggtggttc

SEQ ID NO: 316 - DNA, 52 bp, Artificial Sequence
  Synthetic Polynucleotide
attaagcaataaagcctcagaggccttgatattcacaaacaacggtccacgc

SEQ ID NO: 317 - DNA, 52 bp, Artificial Sequence
  Synthetic Polynucleotide
ctgtagctcaacatgttttaaaatatccagaacaatattacccggtccacgc

SEQ ID NO: 318 - DNA, 52 bp, Artificial Sequence
  Synthetic Polynucleotide
ggcttttgcaaaagaagttttagactttacaaacaattcgacatggtggttc

SEQ ID NO: 319 - DNA, 52 bp, Artificial Sequence
  Synthetic Polynucleotide
aggattagagagtacctttaagtaatttaggcagaggcatttaatagcccga

SEQ ID NO: 320 - DNA, 52 bp, Artificial Sequence
  Synthetic Polynucleotide
aatattcattgaatccccctcgaaacgattttttgtttaacgagagtccact

SEQ ID NO: 321 - DNA, 52 bp, Artificial Sequence
  Synthetic Polynucleotide
aagaggaagcccgaaagacttaatggaaagcgcagtctctgagaaaaaccgt

SEQ ID NO: 322 - DNA, 52 bp, Artificial Sequence
  Synthetic Polynucleotide
accctcgtttaccagacgacgaacgctcatggaaatacctacgaaaaaccgt

SEQ ID NO: 323 - DNA, 52 bp, Artificial Sequence
  Synthetic Polynucleotide
taacggaacaacattattacaagagccgtcaatagataatacagagtccact

SEQ ID NO: 324 - DNA, 52 bp, Artificial Sequence
  Synthetic Polynucleotide
atgtttagactggatagcgtcataaagtaccgacaaaaggtaaatagcccga

SEQ ID NO: 325 - DNA, 52 bp, Artificial Sequence
  Synthetic Polynucleotide
tgaattaccttatgcgattttttacaaaataaacagccatatatggtggttc

SEQ ID NO: 326 - DNA, 52 bp, Artificial Sequence
  Synthetic Polynucleotide
aaacgagaatgaccataaatccatacatggcttttgatgatacggtccacgc

SEQ ID NO: 327 - DNA, 52 bp, Artificial Sequence
  Synthetic Polynucleotide
agatttaggaataccacattcaaatggattatttacattggccggtccacgc

SEQ ID NO: 328 - DNA, 52 bp, Artificial Sequence
  Synthetic Polynucleotide
cgaggcgcagacggtcaatcagttatctaaaatatctttaggatggtggttc

SEQ ID NO: 329 - DNA, 52 bp, Artificial Sequence
  Synthetic Polynucleotide
gtcaggacgttgggaagaaaagacaataaacaacatgttcagaatagcccga

SEQ ID NO: 330 - DNA, 52 bp, Artificial Sequence
  Synthetic Polynucleotide
aggctggctgaccttcatcaataccaacgctaacgagcgtctagagtccact

SEQ ID NO: 331 - DNA, 52 bp, Artificial Sequence
  Synthetic Polynucleotide
taaattgggcttgagatggttttttaacggggtcagtgccttgaaaaaccgt

SEQ ID NO: 332 - DNA, 52 bp, Artificial Sequence
  Synthetic Polynucleotide
tgtgtcgaaatccgcgacctgagtaataaaagggacattctggaaaaaccgt

SEQ ID NO: 333 - DNA, 52 bp, Artificial Sequence
  Synthetic Polynucleotide
tacgaaggcaccaacctaaaactggtcagttggcaaatcaacagagtccact

SEQ ID NO: 334 - DNA, 52 bp, Artificial Sequence
  Synthetic Polynucleotide
ctttgaaagaggacagatgaatatcaacaatagataagtcctaatagcccga

SEQ ID NO: 335 - DNA, 52 bp, Artificial Sequence
  Synthetic Polynucleotide
gtagcaacggctacagaggcttagttgctattttgcacccagatggtggttc

SEQ ID NO: 336 - DNA, 52 bp, Artificial Sequence
  Synthetic Polynucleotide
gatattcattacccaaatcaacagttaatgccccctgcctatcggtccacgc

SEQ ID NO: 337 - DNA, 52 bp, Artificial Sequence
  Synthetic Polynucleotide
ctaaaacactcatctttgaccctgacctgaaagcgtaagaatcggtccacgc

SEQ ID NO: 338 - DNA, 52 bp, Artificial Sequence
  Synthetic Polynucleotide
cgaataataattttttcacgtatcaccttgctgaacctcaaaatggtggttc

SEQ ID NO: 339 - DNA, 52 bp, Artificial Sequence
  Synthetic Polynucleotide
atgaggaagtttccattaaacatcctaatttacgagcatgtaaatagcccga

SEQ ID NO: 340 - DNA, 52 bp, Artificial Sequence
  Synthetic Polynucleotide
ttcgaggtgaatttcttaaacacctcccgacttgcgggaggtagagtccact

SEQ ID NO: 341 - DNA, 52 bp, Artificial Sequence
  Synthetic Polynucleotide
ggatcgtcaccctcagcagcgacatgaaagtattaagaggctgaaaaaccgt

SEQ ID NO: 342 - DNA, 52 bp, Artificial Sequence
  Synthetic Polynucleotide
tttcagcggagtgagaatagatgaatggctattagtctttaagaaaaaccgt

SEQ ID NO: 343 - DNA, 52 bp, Artificial Sequence
  Synthetic Polynucleotide
ctacaacgcctgtagcattccagtgccacgctgagagccagcagagtccact

SEQ ID NO: 344 - DNA, 52 bp, Artificial Sequence
  Synthetic Polynucleotide
ctccaaaaggagcctttaattgtctttccttatcattccaagaatagcccga

SEQ ID NO: 345 - DNA, 52 bp, Artificial Sequence
  Synthetic Polynucleotide
cagagccaccaccctcattttaaggcttatccggtattctaaatggtggttc

SEQ ID NO: 346 - DNA, 52 bp, Artificial Sequence
  Synthetic Polynucleotide
ccgacaatgacaacaaccatctaggattagcggggttttgctcggtccacgc

SEQ ID NO: 347 - DNA, 49 bp, Artificial Sequence
  Synthetic Polynucleotide
tcatcaacattaaaagaacgcgagaaaattgttaaatcagaccgtgcat

SEQ ID NO: 348 - DNA, 42 bp, Artificial Sequence
  Synthetic Polynucleotide
taatcgtaaaactaatcttctgacctaaagctatttttgata

SEQ ID NO: 349 - DNA, 42 bp, Artificial Sequence
  Synthetic Polynucleotide
atatattttaaatggataaataaggcgtaaaaacattatgtc

SEQ ID NO: 350 - DNA, 42 bp, Artificial Sequence
  Synthetic Polynucleotide
gcgagctgaaaaggttactagaaaaagcacgagtagatttct

SEQ ID NO: 351 - DNA, 42 bp, Artificial Sequence
  Synthetic Polynucleotide
ggtcatttttgcggttcttaccagtatattcaaagcgaaccc

SEQ ID NO: 352 - DNA, 42 bp, Artificial Sequence
  Synthetic Polynucleotide
agaaaacgagaatgtgagaatcgccatatttagactggatag

SEQ ID NO: 353 - DNA, 42 bp, Artificial Sequence
  Synthetic Polynucleotide
acgccaaaaggaatagaggcattttcgacggaacaacattag

SEQ ID NO: 354 - DNA, 42 bp, Artificial Sequence
  Synthetic Polynucleotide
tagtaaattgggctacaaaaggtaaagtattcattacccaag

SEQ ID NO: 355 - DNA, 42 bp, Artificial Sequence
  Synthetic Polynucleotide
gaacgaggcgcagaacatgttcagctaaacaaagtacaacca

SEQ ID NO: 356 - DNA, 42 bp, Artificial Sequence
  Synthetic Polynucleotide
ttcatgaggaagttgataagtcctgaactcgtcaccctcatt

SEQ ID NO: 357 - DNA, 42 bp, Artificial Sequence
  Synthetic Polynucleotide
gctttcgaggtgaacgagcatgtagaaaataataattttttg

SEQ ID NO: 358 - DNA, 42 bp, Artificial Sequence
  Synthetic Polynucleotide
tagcgtaacgatcttcattccaagaacgcccatgtaccgtaa

SEQ ID NO: 359 - DNA, 42 bp, Artificial Sequence
  Synthetic Polynucleotide
aagtatagcccggaagaacaagcaagccactcctcaagagca

SEQ ID NO: 360 - DNA, 42 bp, Artificial Sequence
  Synthetic Polynucleotide
atacaggagtgtacccgcgcccaatagcaatcctcattaatc

SEQ ID NO: 361 - DNA, 42 bp, Artificial Sequence
  Synthetic Polynucleotide
caccctcagaaccgggtattctaagaactattagcgtttgac

SEQ ID NO: 362 - DNA, 42 bp, Artificial Sequence
  Synthetic Polynucleotide
cattagcaaggccgtgcgggaggttttgttaaaggtgaattt

SEQ ID NO: 363 - DNA, 42 bp, Artificial Sequence
  Synthetic Polynucleotide
caaagacaccacggttgcacccagctacattaagactcctgg

SEQ ID NO: 364 - DNA, 42 bp, Artificial Sequence
  Synthetic Polynucleotide
agaaacaatgaaatacgagcgtctttccgaattaactgaaaa

SEQ ID NO: 365 - DNA, 28 bp, Artificial Sequence
  Synthetic Polynucleotide
gaacaaacggcggattgacaataattcg

SEQ ID NO: 366 - DNA, 42 bp, Artificial Sequence
  Synthetic Polynucleotide
cgtctggccttcctgtcccggttgataatcagaagagtctgg

SEQ ID NO: 367 - DNA, 42 bp, Artificial Sequence
  Synthetic Polynucleotide
agcaaacaagagaatcaggtaaagattcaaaagtttcaacgc

SEQ ID NO: 368 - DNA, 42 bp, Artificial Sequence
  Synthetic Polynucleotide
aaggataaaaatttttagtagtagcattaacatcaataacct

SEQ ID NO: 369 - DNA, 42 bp, Artificial Sequence
  Synthetic Polynucleotide
gtttagctatattttcctgaatataatgctgtatagagagta

SEQ ID NO: 370 - DNA, 42 bp, Artificial Sequence
  Synthetic Polynucleotide
cctttaattgctccttgtctttaccctgactattcattgaat

SEQ ID NO: 371 - DNA, 42 bp, Artificial Sequence
  Synthetic Polynucleotide
ccccctcaaatgctttaacactatcataacccttaggaatac

SEQ ID NO: 372 - DNA, 42 bp, Artificial Sequence
  Synthetic Polynucleotide
cacattcaactaatgcctttaatcattgtgaattaaggcttg

SEQ ID NO: 373 - DNA, 42 bp, Artificial Sequence
  Synthetic Polynucleotide
ccctgacgagaaacaccgaactgaccaactttgcgaaatccg

SEQ ID NO: 374 - DNA, 42 bp, Artificial Sequence
  Synthetic Polynucleotide
cgacctgctccatgttacgtaatgccactacgaaacggctac

SEQ ID NO: 375 - DNA, 42 bp, Artificial Sequence
  Synthetic Polynucleotide
agaggctttgaggactccgatagttgcgccgacaaaggagcc

SEQ ID NO: 376 - DNA, 42 bp, Artificial Sequence
  Synthetic Polynucleotide
tttaattgtatcggttagacgttagtaaatgaaacgcctgta

SEQ ID NO: 377 - DNA, 42 bp, Artificial Sequence
  Synthetic Polynucleotide
gcattccacagacagccaggaggtttagtaccgccaggcgga

SEQ ID NO: 378 - DNA, 42 bp, Artificial Sequence
  Synthetic Polynucleotide
taagtgccgtcgagagggtcagtgccttgagtaccgttccag

SEQ ID NO: 379 - DNA, 42 bp, Artificial Sequence
  Synthetic Polynucleotide
taagcgtcatacatggcctcagagccgccaccagagccacca

SEQ ID NO: 380 - DNA, 42 bp, Artificial Sequence
  Synthetic Polynucleotide
ccggaaccgcctccctcatcgatagcagcaccgttagagcca

SEQ ID NO: 381 - DNA, 42 bp, Artificial Sequence
  Synthetic Polynucleotide
gcaaaatcaccagtagaatcaatagaaaattcaacatacata

SEQ ID NO: 382 - DNA, 49 bp, Artificial Sequence
  Synthetic Polynucleotide
aaggtggcaacatataaagccctttttaagaaaagaattgagttaagcc

SEQ ID NO: 383 - DNA, 42 bp, Artificial Sequence
  Synthetic Polynucleotide
acaggaagattgaataggaacgccatcaaacgtaatgggata

SEQ ID NO: 384 - DNA, 35 bp, Artificial Sequence
  Synthetic Polynucleotide
agatgggcgcatcgtactcattttttaacctataa

SEQ ID NO: 385 - DNA, 42 bp, Artificial Sequence
  Synthetic Polynucleotide
gcaaatatttaaattgtaaacgtgagatctacaaaggaatca

SEQ ID NO: 386 - DNA, 42 bp, Artificial Sequence
  Synthetic Polynucleotide
ccatcaatatgatattcaaccgtaccctgtaatacttaagaa

SEQ ID NO: 387 - DNA, 42 bp, Artificial Sequence
  Synthetic Polynucleotide
ttagcaaaattaagcaataaagcagtttgaccattagctaaa

SEQ ID NO: 388 - DNA, 42 bp, Artificial Sequence
  Synthetic Polynucleotide
gtacggtgtctggaagtttcattcagaccggaagcaacatca

SEQ ID NO: 389 - DNA, 42 bp, Artificial Sequence
  Synthetic Polynucleotide
aaaagattaagaggaagcccgaaagcgtccaatactgcaaaa

SEQ ID NO: 390 - DNA, 42 bp, Artificial Sequence
  Synthetic Polynucleotide
tagcgagaggcttttgcaaaagaattacaggtagaaagctca

SEQ ID NO: 391 - DNA, 42 bp, Artificial Sequence
  Synthetic Polynucleotide
ttataccagtcaggacgttgggaaatcaacgtaacaaagacc

SEQ ID NO: 392 - DNA, 42 bp, Artificial Sequence
  Synthetic Polynucleotide
aggcgcataggctggctgaccttggagatttgtatcagcaaa

SEQ ID NO: 393 - DNA, 42 bp, Artificial Sequence
  Synthetic Polynucleotide
agaatacactaaaacactcatctgcagcgaaagacagataac

SEQ ID NO: 394 - DNA, 42 bp, Artificial Sequence
  Synthetic Polynucleotide
cgatatattcggtcgctgaggcttcacgttgaaaatccaact

SEQ ID NO: 395 - DNA, 42 bp, Artificial Sequence
  Synthetic Polynucleotide
ttcaacagtttcagcggagtgagaacactgagtttcggaacc

SEQ ID NO: 396 - DNA, 42 bp, Artificial Sequence
  Synthetic Polynucleotide
gccaccctcagagccaccaccctaaggattaggattagcccc

SEQ ID NO: 397 - DNA, 42 bp, Artificial Sequence
  Synthetic Polynucleotide
ctgcctatttcggaacctattatagccagaatggaaagcatt

SEQ ID NO: 398 - DNA, 42 bp, Artificial Sequence
  Synthetic Polynucleotide
gacaggaggttgaggcaggtcagccatcttttcataattgcc

SEQ ID NO: 399 - DNA, 42 bp, Artificial Sequence
  Synthetic Polynucleotide
tttagcgtcagactgtagcgcgttatcaccgtcaccgaaagg

SEQ ID NO: 400 - DNA, 42 bp, Artificial Sequence
  Synthetic Polynucleotide
gcgacattcaaccgattgagggatattacgcagtatgtacca

SEQ ID NO: 401 - DNA, 49 bp, Artificial Sequence
  Synthetic Polynucleotide
gaaggaaaccgaggaaacgcaatcaccctgaacaaagtcagataatatc

SEQ ID NO: 402 - DNA, 42 bp, Artificial Sequence
  Synthetic Polynucleotide
atattttgttaaaattcgcattaaatttctttttcaaatata

SEQ ID NO: 403 - DNA, 42 bp, Artificial Sequence
  Synthetic Polynucleotide
tagctgataaattaatgccggagagggtatttaatggtttga

SEQ ID NO: 404 - DNA, 42 bp, Artificial Sequence
  Synthetic Polynucleotide
cagagcataaagctaaatcggttgtacctaaataagaataaa

SEQ ID NO: 405 - DNA, 42 bp, Artificial Sequence
  Synthetic Polynucleotide
atataacagttgattcccaattctgcgactgtttagtatcat

SEQ ID NO: 406 - DNA, 42 bp, Artificial Sequence
  Synthetic Polynucleotide
acttcaaatatcgcgttttaattcgagcaagccaacgctcaa

SEQ ID NO: 407 - DNA, 42 bp, Artificial Sequence
  Synthetic Polynucleotide
ttttgccagagggggtaatagtaaaatgtttaacaacgccaa

SEQ ID NO: 408 - DNA, 42 bp, Artificial Sequence
  Synthetic Polynucleotide
aaaaatctacgttaataaaacgaactaagccagtaataagag

SEQ ID NO: 409 - DNA, 42 bp, Artificial Sequence
  Synthetic Polynucleotide
tcaagagtaatcttgacaagaaccggataattctgtccagac

SEQ ID NO: 410 - DNA, 42 bp, Artificial Sequence
  Synthetic Polynucleotide
gacccccagcgattataccaagcgcgaatgcagaacgcgcct

SEQ ID NO: 411 - DNA, 42 bp, Artificial Sequence
  Synthetic Polynucleotide
cagggagttaaaggccgcttttgcgggaaagaaaaataatat

SEQ ID NO: 412 - DNA, 42 bp, Artificial Sequence
  Synthetic Polynucleotide
tagaaaggaacaactaaaggaattgcgaccaatcaataatcg

SEQ ID NO: 413 - DNA, 42 bp, Artificial Sequence
  Synthetic Polynucleotide
ttttcagggatagcaagcccaataggaaggtattaaaccaag

SEQ ID NO: 414 - DNA, 42 bp, Artificial Sequence
  Synthetic Polynucleotide
tgaaacatgaaagtattaagaggctgaggtttttattttcat

SEQ ID NO: 415 - DNA, 42 bp, Artificial Sequence
  Synthetic Polynucleotide
gattggccttgatattcacaaacaaataaagcaaatcagata

SEQ ID NO: 416 - DNA, 42 bp, Artificial Sequence
  Synthetic Polynucleotide
tcatcggcattttcggtcatagccccctgcgaggcgttttag

SEQ ID NO: 417 - DNA, 42 bp, Artificial Sequence
  Synthetic Polynucleotide
gaaggtaaatattgacggaaattattcaaagccttaaatcaa

SEQ ID NO: 418 - DNA, 42 bp, Artificial Sequence
  Synthetic Polynucleotide
taacggaatacccaaaagaactggcatgaattttatcctgaa

SEQ ID NO: 419 - DNA, 21 bp, Artificial Sequence
  Synthetic Polynucleotide
cgcattagacgggaagagcct

SEQ ID NO: 420 - DNA, 28 bp, Artificial Sequence
  Synthetic Polynucleotide
aagacaatgtgagcgagtaacaacccgt

SEQ ID NO: 421 - DNA, 42 bp, Artificial Sequence
  Synthetic Polynucleotide
ttttagttaatttcgcatgtcaatcatatgtacagccagctt

SEQ ID NO: 422 - DNA, 42 bp, Artificial Sequence
  Synthetic Polynucleotide
aataccgaccgtgtcaatgcctgagtaatgtgtgatgaacgg

SEQ ID NO: 423 - DNA, 42 bp, Artificial Sequence
  Synthetic Polynucleotide
caccggaatcataatggcatcaattctactaatagaaccctc

SEQ ID NO: 424 - DNA, 42 bp, Artificial Sequence
  Synthetic Polynucleotide
atgcgttatacaaaatggcttagagcttaattgatttggggc

SEQ ID NO: 425 - DNA, 42 bp, Artificial Sequence
  Synthetic Polynucleotide
cagtagggcttaataccataaatcaaaaatcagttgataaga

SEQ ID NO: 426 - DNA, 42 bp, Artificial Sequence
  Synthetic Polynucleotide
catgtaatttaggctacgaggcatagtaagagcaaacagttc

SEQ ID NO: 427 - DNA, 42 bp, Artificial Sequence
  Synthetic Polynucleotide
aatataaagtaccgtgagatggtttaatttcaaagatacata

SEQ ID NO: 428 - DNA, 42 bp, Artificial Sequence
  Synthetic Polynucleotide
gacgacaataaacacggtcaatcataagggaaccagaacgag

SEQ ID NO: 429 - DNA, 42 bp, Artificial Sequence
  Synthetic Polynucleotide
gtttatcaacaatatccattaaacgggtaaaatacttagccg

SEQ ID NO: 430 - DNA, 42 bp, Artificial Sequence
  Synthetic Polynucleotide
cccatcctaatttatttcttaaacagcttgataaaagacttt

SEQ ID NO: 431 - DNA, 42 bp, Artificial Sequence
  Synthetic Polynucleotide
gctgtctttccttaaaagttttgtcgtctttcctatcagctt

SEQ ID NO: 432 - DNA, 42 bp, Artificial Sequence
  Synthetic Polynucleotide
taccgcactcatcgataggtgtatcaccgtactcctcatagt

SEQ ID NO: 433 - DNA, 42 bp, Artificial Sequence
  Synthetic Polynucleotide
cgtaggaatcattatggtaataagttttaacggggttgatat

SEQ ID NO: 434 - DNA, 42 bp, Artificial Sequence
  Synthetic Polynucleotide
tagaaggcttatccccaccctcagagccaccaccttttgatg

SEQ ID NO: 435 - DNA, 42 bp, Artificial Sequence
  Synthetic Polynucleotide
cgaacctcccgactgaaacgtcaccaatgaaaccagagccgc

SEQ ID NO: 436 - DNA, 42 bp, Artificial Sequence
  Synthetic Polynucleotide
gattagttgctattaataagtttattttgtcaccaccattac

SEQ ID NO: 437 - DNA, 42 bp, Artificial Sequence
  Synthetic Polynucleotide
tcttaccaacgctaagcaatagctatcttaccgaaagaaacg

SEQ ID NO: 438 - DNA, 42 bp, Artificial Sequence
  Synthetic Polynucleotide
cggagacagtcactatcaggtcattgcctgaaagccccaaaa

SEQ ID NO: 439 - DNA, 42 bp, Artificial Sequence
  Synthetic Polynucleotide
acaggcaaggcattgcgggagaagcctttaggtgagaaaggc

SEQ ID NO: 440 - DNA, 42 bp, Artificial Sequence
  Synthetic Polynucleotide
ttaaatatgcaaatacatttcgcaaatggtccaataaatcat

SEQ ID NO: 441 - DNA, 42 bp, Artificial Sequence
  Synthetic Polynucleotide
caaagcggattgactccaacaggtcaggatgctcaacatgtt

SEQ ID NO: 442 - DNA, 42 bp, Artificial Sequence
  Synthetic Polynucleotide
gacgataaaaaccggaatcgtcataaatattatagtcagaag

SEQ ID NO: 443 - DNA, 42 bp, Artificial Sequence
  Synthetic Polynucleotide
ttttaagaactggattcatcagttgagattcgtttaccagac

SEQ ID NO: 444 - DNA, 42 bp, Artificial Sequence
  Synthetic Polynucleotide
tgaacggtgtacagctgctcattcagtgaataccttatgcga

SEQ ID NO: 445 - DNA, 42 bp, Artificial Sequence
  Synthetic Polynucleotide
aaaacgaaagagtcgcctgataaattgtgtaaagaggacaga

SEQ ID NO: 446 - DNA, 42 bp, Artificial Sequence
  Synthetic Polynucleotide
catcgcccacgccatcggaacgagggtagcaggcaccaacct

SEQ ID NO: 447 - DNA, 42 bp, Artificial Sequence
  Synthetic Polynucleotide
gattttgctaaatccaaaaaaaaggctccaaatgacaacaac

SEQ ID NO: 448 - DNA, 42 bp, Artificial Sequence
  Synthetic Polynucleotide
ccgccaccctcatcaccagtacaaactacattttctgtatgg

SEQ ID NO: 449 - DNA, 42 bp, Artificial Sequence
  Synthetic Polynucleotide
taaacagttaatgcggggttttgctcagtaccaccctcagaa

SEQ ID NO: 450 - DNA, 42 bp, Artificial Sequence
  Synthetic Polynucleotide
gagccgccgccagcgcagtctctgaatttaacagtgcccgta

SEQ ID NO: 451 - DNA, 42 bp, Artificial Sequence
  Synthetic Polynucleotide
acagaatcaagttcaaaatcaccggaaccagaaccaccacca

SEQ ID NO: 452 - DNA, 42 bp, Artificial Sequence
  Synthetic Polynucleotide
gcgccaaagacaacttgagccatttgggaataatcagtagcg

SEQ ID NO: 453 - DNA, 41 bp, Artificial Sequence
  Synthetic Polynucleotide
ccgaacaaagtttagcaaacgtagaaaattatggtttacca

SEQ ID NO: 454 - DNA, 29 bp, Artificial Sequence
  Synthetic Polynucleotide
agagagataacccacaagtaagcagatag

SEQ ID NO: 455 - DNA, 63 bp, Artificial Sequence
  Synthetic Polynucleotide
agaagatgaaattaactaaaatatatttgaaaaagttttctcgcgttctttgtcttgcgattg

SEQ ID NO: 456 - DNA, 42 bp, Artificial Sequence
  Synthetic Polynucleotide
atttatcacacggtcggtatttcaaaccattaaatttaggtc

SEQ ID NO: 457 - DNA, 42 bp, Artificial Sequence
  Synthetic Polynucleotide
ctagtaattatgattccggtgtttattcttatttaacgcctt

SEQ ID NO: 458 - DNA, 42 bp, Artificial Sequence
  Synthetic Polynucleotide
gtaagaatttgtataacgcatatgatactaaacaggcttttt

SEQ ID NO: 459 - DNA, 42 bp, Artificial Sequence
  Synthetic Polynucleotide
attctcaattaagccctactgttgagcgttggctttatactg

SEQ ID NO: 460 - DNA, 42 bp, Artificial Sequence
  Synthetic Polynucleotide
tgcctctgcctaaattacatgttggcgttgttaaatatggcg

SEQ ID NO: 461 - DNA, 42 bp, Artificial Sequence
  Synthetic Polynucleotide
cttttgtcggtactttatattctcttattactggctcgaaaa

SEQ ID NO: 462 - DNA, 42 bp, Artificial Sequence
  Synthetic Polynucleotide
aacatgttgtttattgtcgtcgtctggacagaattactttac

SEQ ID NO: 463 - DNA, 42 bp, Artificial Sequence
  Synthetic Polynucleotide
acttatctattgttgataaacaggcgcgttctgcattagctg

SEQ ID NO: 464 - DNA, 42 bp, Artificial Sequence
  Synthetic Polynucleotide
atgctcgtaaattaggatgggatattatttttcttgttcagg

SEQ ID NO: 465 - DNA, 42 bp, Artificial Sequence
  Synthetic Polynucleotide
ggaatgataaggaaagacagccgattattgattggtttctac

SEQ ID NO: 466 - DNA, 42 bp, Artificial Sequence
  Synthetic Polynucleotide
ttgttctcgatgagtgcggtacttggtttaatacccgttctt

SEQ ID NO: 467 - DNA, 42 bp, Artificial Sequence
  Synthetic Polynucleotide
ggcgcggtaatgattcctacgatgaaaataaaaacggcttgc

SEQ ID NO: 468 - DNA, 42 bp, Artificial Sequence
  Synthetic Polynucleotide
gaataccggataagccttctatatctgatttgcttgctattg

SEQ ID NO: 469 - DNA, 42 bp, Artificial Sequence
  Synthetic Polynucleotide
tcccgcaagtcgggaggttcgctaaaacgcctcgcgttctta

SEQ ID NO: 470 - DNA, 42 bp, Artificial Sequence
  Synthetic Polynucleotide
ggtgcaaaatagcaactaatcttgatttaaggcttcaaaacc

SEQ ID NO: 471 - DNA, 63 bp, Artificial Sequence
  Synthetic Polynucleotide
gcaaattaggctctggaaagacgctcgttagcgttggtaagattcaggataaaattgtagctg

SEQ ID NO: 472 - DNA, 42 bp, Artificial Sequence
  Synthetic Polynucleotide
attctcaattagcgtggaccgttgagcgttggctttatactg

SEQ ID NO: 473 - DNA, 42 bp, Artificial Sequence
  Synthetic Polynucleotide
tgcctctgcctgaaccaccatttggcgttgttaaatatggcg

SEQ ID NO: 474 - DNA, 42 bp, Artificial Sequence
  Synthetic Polynucleotide
cttttgtcggttcgggctattctcttattactggctcgaaaa

SEQ ID NO: 475 - DNA, 42 bp, Artificial Sequence
  Synthetic Polynucleotide
aacatgttgttagtggactctgtctggacagaattactttac

SEQ ID NO: 476 - DNA, 42 bp, Artificial Sequence
  Synthetic Polynucleotide
acttatctattacggtttttcaggcgcgttctgcattagctg

SEQ ID NO: 477 - DNA, 32 bp, Artificial Sequence
  Synthetic Polynucleotide
taataccataaatcaaaaatcagttgataaga

SEQ ID NO: 478 - DNA, 32 bp, Artificial Sequence
  Synthetic Polynucleotide
aggctacgaggcatagtaagagcaaacagttc

SEQ ID NO: 479 - DNA, 32 bp, Artificial Sequence
  Synthetic Polynucleotide
accgtgagatggtttaatttcaaagatacata

SEQ ID NO: 480 - DNA, 32 bp, Artificial Sequence
  Synthetic Polynucleotide
aacacggtcaatcataagggaaccagaacgag

SEQ ID NO: 481 - DNA, 32 bp, Artificial Sequence
  Synthetic Polynucleotide
aatatccattaaacgggtaaaatacttagccg

SEQ ID NO: 482 - DNA, 42 bp, Artificial Sequence
  Synthetic Polynucleotide
aacggcatctccgtgagcctcctcacagagcctggggtgcct

SEQ ID NO: 483 - DNA, 42 bp, Artificial Sequence
  Synthetic Polynucleotide
ggcagcacccatcccttacactggtgtggttgcgctcactgc

SEQ ID NO: 484 - DNA, 42 bp, Artificial Sequence
  Synthetic Polynucleotide
aaatcccgtggtctggtcagcagcaaccccagctgcattaat

SEQ ID NO: 485 - DNA, 42 bp, Artificial Sequence
  Synthetic Polynucleotide
gagccgccaagcagttgggcggttgtgttttgcgtattgggc

SEQ ID NO: 486 - DNA, 42 bp, Artificial Sequence
  Synthetic Polynucleotide
ggcaccgctaaaacgacggccagtgccaagacgggcaacagc

SEQ ID NO: 487 - DNA, 42 bp, Artificial Sequence
  Synthetic Polynucleotide
cgcgtctgggcctcaggaagatcgcactagagttgcagcaag

SEQ ID NO: 488 - DNA, 42 bp, Artificial Sequence
  Synthetic Polynucleotide
ggagcaaacttttaaccaataggaacgcgaaaatcctgtttg

SEQ ID NO: 489 - DNA, 42 bp, Artificial Sequence
  Synthetic Polynucleotide
gcaaggatatacaaaggctatcaggtcattataaatcaaaag

SEQ ID NO: 490 - DNA, 42 bp, Artificial Sequence
  Synthetic Polynucleotide
ctgtttagctaatacttttgcgggagaatccagtttggaaca

SEQ ID NO: 491 - DNA, 42 bp, Artificial Sequence
  Synthetic Polynucleotide
tacctttaaaccattagatacatttcgccaacgtcaaagggc

SEQ ID NO: 492 - DNA, 42 bp, Artificial Sequence
  Synthetic Polynucleotide
atccccctcggaagcaaactccaacaggactacgtgaaccat

SEQ ID NO: 493 - DNA, 42 bp, Artificial Sequence
  Synthetic Polynucleotide
accacattccaatactgcggaatcgtcagtgccgtaaagcac

SEQ ID NO: 494 - DNA, 42 bp, Artificial Sequence
  Synthetic Polynucleotide
tgccctgacggtagaaagattcatcagtatttagagcttgac

SEQ ID NO: 495 - DNA, 42 bp, Artificial Sequence
  Synthetic Polynucleotide
cgcgacctgcgtaacaaagctgctcattggaagggaagaaag

SEQ ID NO: 496 - DNA, 42 bp, Artificial Sequence
  Synthetic Polynucleotide
acagaggctttgtatcatcgcctgataaaagtgtagcggtca

SEQ ID NO: 497 - DNA, 42 bp, Artificial Sequence
  Synthetic Polynucleotide
cctttaattaaagacagcatcggaacgagcttaatgcgccgc

SEQ ID NO: 498 - DNA, 42 bp, Artificial Sequence
  Synthetic Polynucleotide
tagcattcctgaaaatctccaaaaaaaacgagcacgtataac

SEQ ID NO: 499 - DNA, 42 bp, Artificial Sequence
  Synthetic Polynucleotide
gataagtgcgagtttcgtcaccagtacaagctaaacaggagg

SEQ ID NO: 500 - DNA, 42 bp, Artificial Sequence
  Synthetic Polynucleotide
agtaagcgttaggattagcggggttttggtacgccagaatcc

SEQ ID NO: 501 - DNA, 42 bp, Artificial Sequence
  Synthetic Polynucleotide
caccggaacaatggaaagcgcagtctctcaccgagtaaaaga

SEQ ID NO: 502 - DNA, 42 bp, Artificial Sequence
  Synthetic Polynucleotide
cagcaaaattttcataatcaaaatcacctagcaatacttctt

SEQ ID NO: 503 - DNA, 42 bp, Artificial Sequence
  Synthetic Polynucleotide
taaaggtggcgtcaccgacttgagccattagaagaactcaaa

SEQ ID NO: 504 - DNA, 42 bp, Artificial Sequence
  Synthetic Polynucleotide
attgagttagcagtatgttagcaaacgtcaatattaccgcca

SEQ ID NO: 505 - DNA, 42 bp, Artificial Sequence
  Synthetic Polynucleotide
atttgccagtgagcgctaatatcagagaaaatacctacattt

SEQ ID NO: 506 - DNA, 42 bp, Artificial Sequence
  Synthetic Polynucleotide
tttcatcgttaccaacgctaacgagcgtttacattggcagat

SEQ ID NO: 507 - DNA, 42 bp, Artificial Sequence
  Synthetic Polynucleotide
ccagacgaccgcactcatcgagaacaagggacattctggcca

SEQ ID NO: 508 - DNA, 42 bp, Artificial Sequence
  Synthetic Polynucleotide
aataaacacataaagtaccgacaaaagggcgtaagaatacgt

SEQ ID NO: 509 - DNA, 42 bp, Artificial Sequence
  Synthetic Polynucleotide
atttatcaaaccgaccgtgtgataaatatagtctttaatgcg

SEQ ID NO: 510 - DNA, 42 bp, Artificial Sequence
  Synthetic Polynucleotide
agatgatgattagattaagacgctgagataaaaataccgaac

SEQ ID NO: 511 - DNA, 42 bp, Artificial Sequence
  Synthetic Polynucleotide
agggttagacgaattattcatttcaatttgaggcggtcagta

SEQ ID NO: 512 - DNA, 42 bp, Artificial Sequence
  Synthetic Polynucleotide
agaagtattctgattgtttggattatacgagagccagcagca

SEQ ID NO: 513 - DNA, 42 bp, Artificial Sequence
  Synthetic Polynucleotide
tcatggtcatagccgtgcctgttcttcgcgagatgccgggtt

SEQ ID NO: 514 - DNA, 42 bp, Artificial Sequence
  Synthetic Polynucleotide
acctgcagccagctctttgctcgtcataaagtcggtggtgcc

SEQ ID NO: 515 - DNA, 42 bp, Artificial Sequence
  Synthetic Polynucleotide
atcccacgcaaccaacgtcagcgtggtgctaaaaaaagccgc

SEQ ID NO: 516 - DNA, 42 bp, Artificial Sequence
  Synthetic Polynucleotide
acaggcggccttttctgctcatttgccgcccgggaacggata

SEQ ID NO: 517 - DNA, 42 bp, Artificial Sequence
  Synthetic Polynucleotide
acctcaccggaaacccagtcacgacgttgttctggtgccgga

SEQ ID NO: 518 - DNA, 42 bp, Artificial Sequence
  Synthetic Polynucleotide
aaccaggcaaagcggacgacgacagtatcgccttcctgtagc

SEQ ID NO: 519 - DNA, 42 bp, Artificial Sequence
  Synthetic Polynucleotide
cagctttcatcaatgttaaatcagctcattaagagaatcgat

SEQ ID NO: 520 - DNA, 42 bp, Artificial Sequence
  Synthetic Polynucleotide
gaacggtaatcgtgctatttttgagagatcaaaatttttaga

SEQ ID NO: 521 - DNA, 42 bp, Artificial Sequence
  Synthetic Polynucleotide
accctcatatattaaaacattatgaccctgtatattttcatt

SEQ ID NO: 522 - DNA, 42 bp, Artificial Sequence
  Synthetic Polynucleotide
tggggcgcgagctcgagtagatttagtttgttgctccttttg

SEQ ID NO: 523 - DNA, 42 bp, Artificial Sequence
  Synthetic Polynucleotide
ataagaggtcatttcaaagcgaaccagaccaaatgctttaaa

SEQ ID NO: 524 - DNA, 42 bp, Artificial Sequence
  Synthetic Polynucleotide
cagttcagaaaacttagactggatagcgtcaactaatgcaga

SEQ ID NO: 525 - DNA, 42 bp, Artificial Sequence
  Synthetic Polynucleotide
tacataacgccaaggaacaacattattacagagaaacaccag

SEQ ID NO: 526 - DNA, 42 bp, Artificial Sequence
  Synthetic Polynucleotide
aacgagtagtaaattcattacccaaatcaactccatgttact

SEQ ID NO: 527 - DNA, 42 bp, Artificial Sequence
  Synthetic Polynucleotide
tagccggaacgagcaaagtacaacggagatttgaggactaaa

SEQ ID NO: 528 - DNA, 42 bp, Artificial Sequence
  Synthetic Polynucleotide
gactttttcatgacgtcaccctcagcagcggtatcggtttat

SEQ ID NO: 529 - DNA, 42 bp, Artificial Sequence
  Synthetic Polynucleotide
cagcttgctttcgtaataattttttcacgtacagacagccct

SEQ ID NO: 530 - DNA, 42 bp, Artificial Sequence
  Synthetic Polynucleotide
catagttagcgtaccatgtaccgtaacactcgtcgagagggt

SEQ ID NO: 531 - DNA, 42 bp, Artificial Sequence
  Synthetic Polynucleotide
tgatataagtatactcctcaagagaaggatcatacatggctt

SEQ ID NO: 532 - DNA, 42 bp, Artificial Sequence
  Synthetic Polynucleotide
ttgatgatacaggatcctcattaaagccagcgcctccctcag

SEQ ID NO: 533 - DNA, 42 bp, Artificial Sequence
  Synthetic Polynucleotide
agccgccaccctcattagcgtttgccatctcaccagtagcac

SEQ ID NO: 534 - DNA, 42 bp, Artificial Sequence
  Synthetic Polynucleotide
cattaccattagctaaaggtgaattatcaccaacatataaaa

SEQ ID NO: 535 - DNA, 42 bp, Artificial Sequence
  Synthetic Polynucleotide
gaaacgcaaagacttaagactccttattacagcccaataata

SEQ ID NO: 536 - DNA, 42 bp, Artificial Sequence
  Synthetic Polynucleotide
agagcaagaaacacaaagtcagagggtaatttacaaaataaa

SEQ ID NO: 537 - DNA, 42 bp, Artificial Sequence
  Synthetic Polynucleotide
cagccatattattaattttatcctgaatctaggaatcattac

SEQ ID NO: 538 - DNA, 42 bp, Artificial Sequence
  Synthetic Polynucleotide
cgcgcccaatagcggtattaaaccaagtacgacaataaacaa

SEQ ID NO: 539 - DNA, 42 bp, Artificial Sequence
  Synthetic Polynucleotide
catgttcagctaagccagtaataagagaatcggaatcataat

SEQ ID NO: 540 - DNA, 42 bp, Artificial Sequence
  Synthetic Polynucleotide
tactagaaaaagcatttaatggtttgaaataatcataggtct

SEQ ID NO: 541 - DNA, 42 bp, Artificial Sequence
  Synthetic Polynucleotide
gagagactaccttgaaaacatagcgatagcaacaaacatcaa

SEQ ID NO: 542 - DNA, 42 bp, Artificial Sequence
  Synthetic Polynucleotide
gaaaacaaaattaacaaaatcgcgcagaggacctaccatatc

SEQ ID NO: 543 - DNA, 46 bp, Artificial Sequence
  Synthetic Polynucleotide
aaaattatttgcaaattcatcaatataatcagactttacaaacaat

SEQ ID NO: 544 - DNA, 49 bp, Artificial Sequence
  Synthetic Polynucleotide
tcgacaactctaacaactaatcgtcaatagataatgaacctcaaatatc

SEQ ID NO: 545 - DNA, 33 bp, Artificial Sequence
  Synthetic Polynucleotide
tctgccagcacgtgtttcctgtgtgccgctcac

SEQ ID NO: 546 - DNA, 42 bp, Artificial Sequence
  Synthetic Polynucleotide
tgggtaaaggttggtgccggtgccccctgcataccgggggtt

SEQ ID NO: 547 - DNA, 42 bp, Artificial Sequence
  Synthetic Polynucleotide
ccggacttgtagagcttacggctggaggtgtgcggctggtaa

SEQ ID NO: 548 - DNA, 42 bp, Artificial Sequence
  Synthetic Polynucleotide
caaacttaaattagtgatgaagggtaaagttaacggaacgtg

SEQ ID NO: 549 - DNA, 42 bp, Artificial Sequence
  Synthetic Polynucleotide
cgccagggttttcaatcggcgaaacgtacagaaacagcggat

SEQ ID NO: 550 - DNA, 42 bp, Artificial Sequence
  Synthetic Polynucleotide
gccagtttgagggccattcgccattcaggctaagttgggtaa

SEQ ID NO: 551 - DNA, 42 bp, Artificial Sequence
  Synthetic Polynucleotide
gcattaaattttcattaaatgtgagcgagtaaccgtgcatct

SEQ ID NO: 552 - DNA, 42 bp, Artificial Sequence
  Synthetic Polynucleotide
ccggagagggtaaaaactagcatgtcaatcttgttaaaattc

SEQ ID NO: 553 - DNA, 42 bp, Artificial Sequence
  Synthetic Polynucleotide
tcggttgtaccattaaatgcaatgcctgaggataaattaatg

SEQ ID NO: 554 - DNA, 42 bp, Artificial Sequence
  Synthetic Polynucleotide
caattctgcgaagaaaaggtggcatcaattcataaagctaaa

SEQ ID NO: 555 - DNA, 42 bp, Artificial Sequence
  Synthetic Polynucleotide
ttaattcgagcttttgcggatggcttagagacagttgattcc

SEQ ID NO: 556 - DNA, 42 bp, Artificial Sequence
  Synthetic Polynucleotide
atagtaaaatgtgagaatgaccataaatcaaaatatcgcgtt

SEQ ID NO: 557 - DNA, 42 bp, Artificial Sequence
  Synthetic Polynucleotide
aaacgaactaacaaggaattacgaggcataccagagggggta

SEQ ID NO: 558 - DNA, 42 bp, Artificial Sequence
  Synthetic Polynucleotide
aagaaccggatattgggcttgagatggttttctacgttaata

SEQ ID NO: 559 - DNA, 42 bp, Artificial Sequence
  Synthetic Polynucleotide
ccaagcgcgaaagcgcagacggtcaatcatagtaatcttgac

SEQ ID NO: 560 - DNA, 42 bp, Artificial Sequence
  Synthetic Polynucleotide
cttttgcgggatggaagtttccattaaacgccagcgattata

SEQ ID NO: 561 - DNA, 42 bp, Artificial Sequence
  Synthetic Polynucleotide
aggaattgcgaaaggtgaatttcttaaacaagttaaaggccg

SEQ ID NO: 562 - DNA, 42 bp, Artificial Sequence
  Synthetic Polynucleotide
cccaataggaacacgatctaaagttttgtcaggaacaactaa

SEQ ID NO: 563 - DNA, 42 bp, Artificial Sequence
  Synthetic Polynucleotide
aagaggctgagagcccggaataggtgtatcagggatagcaag

SEQ ID NO: 564 - DNA, 42 bp, Artificial Sequence
  Synthetic Polynucleotide
acaaacaaataaagtgtactggtaataagtcatgaaagtatt

SEQ ID NO: 565 - DNA, 42 bp, Artificial Sequence
  Synthetic Polynucleotide
catagcccccttagaaccgccaccctcagagccttgatattc

SEQ ID NO: 566 - DNA, 42 bp, Artificial Sequence
  Synthetic Polynucleotide
gaaattattcataaggccggaaacgtcaccggcattttcggt

SEQ ID NO: 567 - DNA, 42 bp, Artificial Sequence
  Synthetic Polynucleotide
gaactggcatgaaccacggaataagtttattaaatattgacg

SEQ ID NO: 568 - DNA, 42 bp, Artificial Sequence
  Synthetic Polynucleotide
gaacaccctgaaatgaaatagcaatagctagaatacccaaaa

SEQ ID NO: 569 - DNA, 42 bp, Artificial Sequence
  Synthetic Polynucleotide
gcacccagctactatcccaatccaaataagggagaattaact

SEQ ID NO: 570 - DNA, 42 bp, Artificial Sequence
  Synthetic Polynucleotide
attccaagaacgaagcaaatcagatatagaagttgctatttt

SEQ ID NO: 571 - DNA, 42 bp, Artificial Sequence
  Synthetic Polynucleotide
aggcattttcgatgcagaacgcgcctgttttctttccttatc

SEQ ID NO: 572 - DNA, 42 bp, Artificial Sequence
  Synthetic Polynucleotide
cttctgacctaactgtttagtatcatatgctaatttaggcag

SEQ ID NO: 573 - DNA, 42 bp, Artificial Sequence
  Synthetic Polynucleotide
cttagaatcctttttaacctccggcttaggagttaatttcat

SEQ ID NO: 574 - DNA, 42 bp, Artificial Sequence
  Synthetic Polynucleotide
gaataccaagttattacatttaacaatttcaattaattttcc

SEQ ID NO: 575 - DNA, 42 bp, Artificial Sequence
  Synthetic Polynucleotide
tcagatgatggccgtaaaacagaaataaagcctgattgcttt

SEQ ID NO: 576 - DNA, 42 bp, Artificial Sequence
  Synthetic Polynucleotide
tctttaggagcacgtattaaatcctttgcctattcctgatta

SEQ ID NO: 577 - DNA, 42 bp, Artificial Sequence
  Synthetic Polynucleotide
aattccacacaagggccgttttcacggtcatcagacgatcca

SEQ ID NO: 578 - DNA, 42 bp, Artificial Sequence
  Synthetic Polynucleotide
gcgcagtgtcacccgggtcactgttgccctccagcatcagcg

SEQ ID NO: 579 - DNA, 42 bp, Artificial Sequence
  Synthetic Polynucleotide
gggtcattgcaggccagagcacatcctcataaacgatgctga

SEQ ID NO: 580 - DNA, 42 bp, Artificial Sequence
  Synthetic Polynucleotide
ttgccgttccggacggaaaaagagacgcagcgccatgtttac

SEQ ID NO: 581 - DNA, 42 bp, Artificial Sequence
  Synthetic Polynucleotide
cagtcccggaatatgtgctgcaaggcgattgcgcaactgttg

SEQ ID NO: 582 - DNA, 42 bp, Artificial Sequence
  Synthetic Polynucleotide
ggaagggcgatcgtagatgggcgcatcgtaacaacccgtcgg

SEQ ID NO: 583 - DNA, 42 bp, Artificial Sequence
  Synthetic Polynucleotide
attctccgtgggttgtaaacgttaatattatatgtaccccgg

SEQ ID NO: 584 - DNA, 42 bp, Artificial Sequence
  Synthetic Polynucleotide
ttgataatcagaattcaaccgttctagcttaatgtgtaggta

SEQ ID NO: 585 - DNA, 42 bp, Artificial Sequence
  Synthetic Polynucleotide
aagattcaaaaggcaataaagcctcagagctactaatagtag

SEQ ID NO: 586 - DNA, 42 bp, Artificial Sequence
  Synthetic Polynucleotide
tagcattaacataagtttcattccatatacttaattgctgaa

SEQ ID NO: 587 - DNA, 42 bp, Artificial Sequence
  Synthetic Polynucleotide
tataatgctgtagaagcccgaaagacttcaaaatcaggtctt

SEQ ID NO: 588 - DNA, 42 bp, Artificial Sequence
  Synthetic Polynucleotide
taccctgactatttgcaaaagaagttttggtaagagcaacac

SEQ ID NO: 589 - DNA, 42 bp, Artificial Sequence
  Synthetic Polynucleotide
tatcataaccctgacgttgggaagaaaaaaatttcaacttta

SEQ ID NO: 590 - DNA, 42 bp, Artificial Sequence
  Synthetic Polynucleotide
atcattgtgaatggctgaccttcatcaagaagggaaccgaac

SEQ ID NO: 591 - DNA, 42 bp, Artificial Sequence
  Synthetic Polynucleotide
tgaccaactttgacactcatctttgacccggtaaaatacgta

SEQ ID NO: 592 - DNA, 42 bp, Artificial Sequence
  Synthetic Polynucleotide
atgccactacgacgctgaggcttgcaggggcttgataccgat

SEQ ID NO: 593 - DNA, 42 bp, Artificial Sequence
  Synthetic Polynucleotide
agttgcgccgacgcggagtgagaatagaagtctttccagacg

SEQ ID NO: 594 - DNA, 42 bp, Artificial Sequence
  Synthetic Polynucleotide
ttagtaaatgaaccaccaccctcattttcaccgtactcagga

SEQ ID NO: 595 - DNA, 42 bp, Artificial Sequence
  Synthetic Polynucleotide
ggtttagtaccgaacctattattctgaaatttaacggggtca

SEQ ID NO: 596 - DNA, 42 bp, Artificial Sequence
  Synthetic Polynucleotide
gtgccttgagtaggcaggtcagacgattggccaccaccctca

SEQ ID NO: 597 - DNA, 42 bp, Artificial Sequence
  Synthetic Polynucleotide
gagccgccaccatgtagcgcgttttcatcaatgaaaccatcg

SEQ ID NO: 598 - DNA, 42 bp, Artificial Sequence
  Synthetic Polynucleotide
atagcagcaccggattgagggagggaaggtttgtcacaatca

SEQ ID NO: 599 - DNA, 42 bp, Artificial Sequence
  Synthetic Polynucleotide
atagaaaattcagaaacgcaataataacgtcttaccgaagcc

SEQ ID NO: 600 - DNA, 42 bp, Artificial Sequence
  Synthetic Polynucleotide
ctttttaagaaagggaagcgcattagacgaaacgattttttg

SEQ ID NO: 601 - DNA, 42 bp, Artificial Sequence
  Synthetic Polynucleotide
tttaacgtcaaaagccttaaatcaagattaggcttatccggt

SEQ ID NO: 602 - DNA, 42 bp, Artificial Sequence
  Synthetic Polynucleotide
attctaagaacgcaatcaataatcggctgatcaacaatagat

SEQ ID NO: 603 - DNA, 42 bp, Artificial Sequence
  Synthetic Polynucleotide
aagtcctgaacattaacaacgccaacatggttatacaaattc

SEQ ID NO: 604 - DNA, 42 bp, Artificial Sequence
  Synthetic Polynucleotide
ttaccagtataatttttcaaatatattttttgggttatataa

SEQ ID NO: 605 - DNA, 42 bp, Artificial Sequence
  Synthetic Polynucleotide
ctatatgtaaattgtaaatcgtcgctattatttgaattacct

SEQ ID NO: 606 - DNA, 42 bp, Artificial Sequence
  Synthetic Polynucleotide
tttttaatggaaaaacaataacggattcgaaattgcgtagat

SEQ ID NO: 607 - DNA, 42 bp, Artificial Sequence
  Synthetic Polynucleotide
tttcaggtttaagagcggaattatcatcacgaacgttattaa

SEQ ID NO: 608 - DNA, 31 bp, Artificial Sequence
  Synthetic Polynucleotide
ttttaaaagtttaaaggaattgagtaaaata

SEQ ID NO: 609 - DNA, 32 bp, Artificial Sequence
  Synthetic Polynucleotide
cggaagcataaagtgtaattgaggatccccgg

SEQ ID NO: 610 - DNA, 42 bp, Artificial Sequence
  Synthetic Polynucleotide
gtgcactctgtggtctcacattaattgcttcagcaaatcgtt

SEQ ID NO: 611 - DNA, 42 bp, Artificial Sequence
  Synthetic Polynucleotide
cactcaatccgccgggaaacctgtcgtggcaagaatgccaac

SEQ ID NO: 612 - DNA, 42 bp, Artificial Sequence
  Synthetic Polynucleotide
tccgttttttcgtcgcggggagaggcggacatcgacataaaa

SEQ ID NO: 613 - DNA, 42 bp, Artificial Sequence
  Synthetic Polynucleotide
atagactttctccgtcttttcaccagtgagctttcagaggtg

SEQ ID NO: 614 - DNA, 42 bp, Artificial Sequence
  Synthetic Polynucleotide
ctcttcgctattaccgcctggccctgagccagccagctttcc

SEQ ID NO: 615 - DNA, 42 bp, Artificial Sequence
  Synthetic Polynucleotide
cggattgaccgtaattgccccagcaggccatcaaaaataatt

SEQ ID NO: 616 - DNA, 42 bp, Artificial Sequence
  Synthetic Polynucleotide
aaaacaggaagattatcggcaaaatcccttgcctgagagtct

SEQ ID NO: 617 - DNA, 42 bp, Artificial Sequence
  Synthetic Polynucleotide
ggccggagacagtcgggttgagtgttgtgcctttatttcaac

SEQ ID NO: 618 - DNA, 42 bp, Artificial Sequence
  Synthetic Polynucleotide
catacaggcaaggcaagaacgtggactcaaatggtcaataac

SEQ ID NO: 619 - DNA, 42 bp, Artificial Sequence
  Synthetic Polynucleotide
gttttaaatatgcacagggcgatggccctcaggattagagag

SEQ ID NO: 620 - DNA, 42 bp, Artificial Sequence
  Synthetic Polynucleotide
aagcaaagcggatttttttggggtcgagtaaatattcattga

SEQ ID NO: 621 - DNA, 42 bp, Artificial Sequence
  Synthetic Polynucleotide
gacgacgataaaaaaaagggagcccccgtgagatttaggaat

SEQ ID NO: 622 - DNA, 42 bp, Artificial Sequence
  Synthetic Polynucleotide
cgattttaagaactaacgtggcgagaaacagtgaataaggct

SEQ ID NO: 623 - DNA, 42 bp, Artificial Sequence
  Synthetic Polynucleotide
agatgaacggtgtagctagggcgctggcattgtgtcgaaatc

SEQ ID NO: 624 - DNA, 42 bp, Artificial Sequence
  Synthetic Polynucleotide
cctaaaacgaaagaaccacacccgccgcgggtagcaacggct

SEQ ID NO: 625 - DNA, 42 bp, Artificial Sequence
  Synthetic Polynucleotide
aaccatcgcccacgtatggttgctttgaggctccaaaaggag

SEQ ID NO: 626 - DNA, 42 bp, Artificial Sequence
  Synthetic Polynucleotide
tgggattttgctaaagaatcagagcgggaactacaacgcctg

SEQ ID NO: 627 - DNA, 42 bp, Artificial Sequence
  Synthetic Polynucleotide
gaaccgccaccctctttagacaggaacgctcagtaccaggcg

SEQ ID NO: 628 - DNA, 42 bp, Artificial Sequence
  Synthetic Polynucleotide
gtataaacagttaaataatcagtgaggcgaatttaccgttcc

SEQ ID NO: 629 - DNA, 42 bp, Artificial Sequence
  Synthetic Polynucleotide
ccagagccgccgcccaaattaaccgttgggaaccagagccac

SEQ ID NO: 630 - DNA, 42 bp, Artificial Sequence
  Synthetic Polynucleotide
gcgacagaatcaagatcacttgcctgagttgggaattagagc

SEQ ID NO: 631 - DNA, 42 bp, Artificial Sequence
  Synthetic Polynucleotide
ccagcgccaaagacggtaatatccagaaagaaaatacataca

SEQ ID NO: 632 - DNA, 42 bp, Artificial Sequence
  Synthetic Polynucleotide
atagccgaacaaagaaaaacgctcatgggataacccacaaga

SEQ ID NO: 633 - DNA, 42 bp, Artificial Sequence
  Synthetic Polynucleotide
agcagcctttacagctgaaatggattatctttccagagccta

SEQ ID NO: 634 - DNA, 42 bp, Artificial Sequence
  Synthetic Polynucleotide
ttagcgaacctcccaccagtaataaaagcaagccgtttttat

SEQ ID NO: 635 - DNA, 42 bp, Artificial Sequence
  Synthetic Polynucleotide
atatcccatcctaacttctgacctgaaataaagtaattctgt

SEQ ID NO: 636 - DNA, 42 bp, Artificial Sequence
  Synthetic Polynucleotide
tcaacagtagggctttttgaatggctataggcgttaaataag

SEQ ID NO: 637 - DNA, 42 bp, Artificial Sequence
  Synthetic Polynucleotide
aatccaatcgcaagtaaaacatcgccatagagtcaatagtga

SEQ ID NO: 638 - DNA, 42 bp, Artificial Sequence
  Synthetic Polynucleotide
aaatcaatatatgtagataaaacagaggacctgagcaaaaga

SEQ ID NO: 639 - DNA, 42 bp, Artificial Sequence
  Synthetic Polynucleotide
aatatacagtaacaaacagtgccacgctttctgaataatgga

SEQ ID NO: 640 - DNA, 42 bp, Artificial Sequence
  Synthetic Polynucleotide
tatcattttgcggaagcatcaccttgctacatttgaggattt

SEQ ID NO: 641 - DNA, 42 bp, Artificial Sequence
  Synthetic Polynucleotide
aatgagtgagctaagctgcggccagaatgcggccatacgagc

SEQ ID NO: 642 - DNA, 42 bp, Artificial Sequence
  Synthetic Polynucleotide
ccgctttccagtcgggcgcggttgcggtatgagtgcgcgcct

SEQ ID NO: 643 - DNA, 42 bp, Artificial Sequence
  Synthetic Polynucleotide
gaatcggccaacgctcgtcgctggcagcctccggcgctttcg

SEQ ID NO: 644 - DNA, 42 bp, Artificial Sequence
  Synthetic Polynucleotide
gccagggtggtttttggtgaagggatagctctccaaacgcgg

SEQ ID NO: 645 - DNA, 42 bp, Artificial Sequence
  Synthetic Polynucleotide
tgattgcccttcacgccagctggcgaaagggggttgtgagag

SEQ ID NO: 646 - DNA, 42 bp, Artificial Sequence
  Synthetic Polynucleotide
cggtccacgctggttgggataggtcacgttggtggtgcgggc

SEQ ID NO: 647 - DNA, 42 bp, Artificial Sequence
  Synthetic Polynucleotide
atggtggttccgaagtataagcaaatatttaaaaacaaacgg

SEQ ID NO: 648 - DNA, 42 bp, Artificial Sequence
  Synthetic Polynucleotide
aatagcccgagataaaatcaccatcaatatgataaagcccca

SEQ ID NO: 649 - DNA, 42 bp, Artificial Sequence
  Synthetic Polynucleotide
agagtccactattaaaagaattagcaaaattaaggtgagaaa

SEQ ID NO: 650 - DNA, 42 bp, Artificial Sequence
  Synthetic Polynucleotide
gaaaaaccgtctatactaaagtacggtgtctggccaataaat

SEQ ID NO: 651 - DNA, 42 bp, Artificial Sequence
  Synthetic Polynucleotide
cacccaaatcaagtgcatcaaaaagattaagaggctcaacat

SEQ ID NO: 652 - DNA, 42 bp, Artificial Sequence
  Synthetic Polynucleotide
taaatcggaaccctccaaaatagcgagaggctttatagtcag

SEQ ID NO: 653 - DNA, 42 bp, Artificial Sequence
  Synthetic Polynucleotide
ggggaaagccggcgggctcattataccagtcagcgtttacca

SEQ ID NO: 654 - DNA, 42 bp, Artificial Sequence
  Synthetic Polynucleotide
cgaaaggagcgggccagaccaggcgcataggcttaccttatg

SEQ ID NO: 655 - DNA, 42 bp, Artificial Sequence
  Synthetic Polynucleotide
cgctgcgcgtaaccggcaaaagaatacactaaaaaagaggac

SEQ ID NO: 656 - DNA, 42 bp, Artificial Sequence
  Synthetic Polynucleotide
tacagggcgcgtaccataaccgatatattcggtaggcaccaa

SEQ ID NO: 657 - DNA, 42 bp, Artificial Sequence
  Synthetic Polynucleotide
gtgctttcctcgttacaactttcaacagtttcaaatgacaac

SEQ ID NO: 658 - DNA, 42 bp, Artificial Sequence
  Synthetic Polynucleotide
ccgattaaagggatagaaccgccaccctcagagttttctgta

SEQ ID NO: 659 - DNA, 42 bp, Artificial Sequence
  Synthetic Polynucleotide
tgagaagtgttttttgccccctgcctatttcggccaccctca

SEQ ID NO: 660 - DNA, 42 bp, Artificial Sequence
  Synthetic Polynucleotide
gtctgtccatcacgagcattgacaggaggttgaacagtgccc

SEQ ID NO: 661 - DNA, 42 bp, Artificial Sequence
  Synthetic Polynucleotide
tgattagtaataactttgcctttagcgtcagacgaaccacca

SEQ ID NO: 662 - DNA, 42 bp, Artificial Sequence
  Synthetic Polynucleotide
ctatcggccttgctaaaagggcgacattcaacctaatcagta

SEQ ID NO: 663 - DNA, 42 bp, Artificial Sequence
  Synthetic Polynucleotide
gccattgcaacaggttaccagaaggaaaccgagtatggttta

SEQ ID NO: 664 - DNA, 42 bp, Artificial Sequence
  Synthetic Polynucleotide
tgacgctcaatcgtagagaataacataaaaacaagtaagcag

SEQ ID NO: 665 - DNA, 42 bp, Artificial Sequence
  Synthetic Polynucleotide
tcaccagtcacacggacttgcgggaggttttgaaatgaaaat

SEQ ID NO: 666 - DNA, 42 bp, Artificial Sequence
  Synthetic Polynucleotide
acagagatagaacctttacgagcatgtagaaaccgaggcgtt

SEQ ID NO: 667 - DNA, 42 bp, Artificial Sequence
  Synthetic Polynucleotide
ggcacagacaatattaattgagaatcgccatatagaaaaata

SEQ ID NO: 668 - DNA, 42 bp, Artificial Sequence
  Synthetic Polynucleotide
cgaactgatagcccacaaagaacgcgagaaaacagccaacgc

SEQ ID NO: 669 - DNA, 42 bp, Artificial Sequence
  Synthetic Polynucleotide
gaaccaccagcagagagtgaataaccttgcttcgctgatgca

SEQ ID NO: 670 - DNA, 42 bp, Artificial Sequence
  Synthetic Polynucleotide
ttaacaccgcctgcgtaccttttacatcgggagacagtacat

SEQ ID NO: 671 - DNA, 42 bp, Artificial Sequence
  Synthetic Polynucleotide
aatgaaaaatctaaacaaagaaaccaccagaagcgtcagatg

SEQ ID NO: 672 - DNA, 42 bp, Artificial Sequence
  Synthetic Polynucleotide
aaaccctcaatcaagttggcaaatcaacagttggagtaacat

SEQ ID NO: 673 - DNA, 35 bp, Artificial Sequence
  Synthetic Polynucleotide
cgctggttgggataggtcacgttggtggtgcgggc

SEQ ID NO: 674 - DNA, 35 bp, Artificial Sequence
  Synthetic Polynucleotide
ttccgaagtataagcaaatatttaaaaacaaacgg

SEQ ID NO: 675 - DNA, 35 bp, Artificial Sequence
  Synthetic Polynucleotide
cgagataaaatcaccatcaatatgataaagcccca

SEQ ID NO: 676 - DNA, 35 bp, Artificial Sequence
  Synthetic Polynucleotide
actattaaaagaattagcaaaattaaggtgagaaa

SEQ ID NO: 677 - DNA, 35 bp, Artificial Sequence
  Synthetic Polynucleotide
cgtctatactaaagtacggtgtctggccaataaat

SEQ ID NO: 678 - DNA, 32 bp, Artificial Sequence
  Synthetic Polynucleotide
tggttgggataggtcacgttggtggtgcgggc

SEQ ID NO: 679 - DNA, 32 bp, Artificial Sequence
  Synthetic Polynucleotide
cgaagtataagcaaatatttaaaaacaaacgg

SEQ ID NO: 680 - DNA, 32 bp, Artificial Sequence
  Synthetic Polynucleotide
gataaaatcaccatcaatatgataaagcccca

SEQ ID NO: 681 - DNA, 32 bp, Artificial Sequence
  Synthetic Polynucleotide
attaaaagaattagcaaaattaaggtgagaaa

SEQ ID NO: 682 - DNA, 32 bp, Artificial Sequence
  Synthetic Polynucleotide
ctatactaaagtacggtgtctggccaataaat

SEQ ID NO: 683 - DNA, 62 bp, Artificial Sequence
  Synthetic Polynucleotide
tgcaatttaattcttttagcatttcaatatttgtagatttgagaatttcgtttttttattca

SEQ ID NO: 684 - DNA, 84 bp, Artificial Sequence
  Synthetic Polynucleotide
tggttctggagttttactcgggacacttcagcgtaatatcggaagcaggcactttgaaacctataagtcctgactattaataac

SEQ ID NO: 685 - DNA, 40 bp, Artificial Sequence
  Synthetic Polynucleotide
ggctccctttagggttccgatgatcctcaactgtgaggag

SEQ ID NO: 686 - DNA, 40 bp, Artificial Sequence
  Synthetic Polynucleotide
ctcctcacagttgaggatcatcggaaccctaaagggagcc

SEQ ID NO: 687 - DNA, 26 bp, Artificial Sequence
  Synthetic Polynucleotide
  misc_feature (9)..(17): n is a, c, g, or t
gcctggggnnnnnnnnntgagtgagc

SEQ ID NO: 688 - DNA, 27 bp, Artificial Sequence
  Synthetic Polynucleotide
  misc_feature (11)..(19): n is a, c, g, or t
agctcactcannnnnnnnnccccaggc